European Patent Application EP 4 541 902 A1, published April 23, 2025. Title: Method for producing 4-(aminomethyl)cyclohexane-1-carboxylic acid. Applicant: キリンホールディングス株式会社. The sequence listing filed with the application follows.

SEQUENCE LISTING (200 sequences)

SEQ ID NO: 1 - protein, 453 aa, Pseudomonas putida KT2440
MSVNNPQTREWQTLSGEHHLAPFSDYKQLKEKGPRIITKAQGVHLWDSEGHKILDGMAGLWCVAVGYGREELVQAAEKQMRELPYYNLFFQTAHPPALELAKAITDVAPKGMTHVFFTGSGSEGNDTVLRMVRHYWALKGKPHKQTIIGRINGYHGSTFAGACLGGMSGMHEQGGLPIPGIVHIPQPYWFGEGGDMTPDEFGVWAAEQLEKKILEVGEDNVAAFIAEPIQGAGGVIIPPETYWPKVKEILARYDILFVADEVICGFGRTGEWFGSDYYDLKPDLMTIAKGLTSGYIPMGGVIVRDTVAKVISEGGDFNHGFTYSGHPVAAAVGLENLRILRDEKIVEKARTEAAPYLQKRLRELQDHPLVGEVRGLGMLGAIELVKDKATRSRYEGKGVGMICRTFCFENGLIMRAVGDTMIIAPPLVISHAEIDELVEKARKCLDLTLEAIQ

SEQ ID NO: 2 - protein, 460 aa, Pseudomonas putida KT2440
MNAPFAPQRQTRDYQAADAAHHIHAFLDQKALNAEGPRVIVGGERLHLWDSEGKRYLDGMSGLWCTQLGYGRRDLTAAAATQMDQLAYYNMFFHTTHPAVIELSELLFSLLPGHYSHAIYTNSGSEANEVLIRTVRRYWQVVGQPGKKIMIGRWNGYHGSTLAATALGGMKFMHDMGGLIPDVAHIDEPYWYAEGGELTPAEFGRRCALQLEEKILELGAENVAGFIAEPFQGAGGMIFPPESYWPEIQRICRQYDVLLCADEVIGGFGRTGEWFAHEYFGFEPDTLSIAKGLTSGYVPMGGLVLSKRIAEALVERGGVFAHGLTYSGHPVAAAVAIANLKALRDEGIVRQVKDDTGPYLQRILREVFADHPLIGQVQGAGLVAALQFAEHKPTRKRFANENDLAWQCRTFGFEEGVIIRSTLGRMIMAPALIANHSELDELVEKTRIAVDRTARLVGKL

SEQ ID NO: 3 - protein, 453 aa, Aeromonas salmonicida subsp. salmonicida
MQHTTREWQQLDASHHLHPFTDFQALNQKGSRIITRAEGIYLEDSDGRRILDGMAGLWCVNMGYGRQELVEAATKQMQQLPYYNLFFQTAHPPVIELATLLAEVTPSHLNHVFFTGSGSECNDTVLRMVRHYWASKGQPDKQVIISRHNAYHGSTVAGASLGGMKGMHAQGGLPIPGIVHIDQPYHFGEGQGMSAHEFGLERARQLEQKILELGVDKVAAFIGEPIQGAGGVIIPPDSYWPEIQRICDKYGILLIADEVICGFGRTGHWFASEGFGIKPDLMCLAKGITSGYLPMGAVMVGDRVARVLVEEGGEFNHGFTYSGHPVACAVAIANIKLMQSESIVKRIHDTIGPYLQRRWRELADHPLVGETRGKGLVAALEIVQDKQTNSRFPAGLQAGMTCREFCFNNGLVMRAVGDTMIISPPLVITEEQVDELVNLARLSLDLTAAKLKG

SEQ ID NO: 4 - protein, 459 aa, Escherichia coli K12 MG1655
MNRLPSSASALACSAHALNLIEKRTLDHEEMKALNREVIEYFKEHVNPGFLEYRKSVTAGGDYGAVEWQAGSLNTLVDTQGQEFIDCLGGFGIFNVGHRNPVVVSAVQNQLAKQPLHSQELLDPLRAMLAKTLAALTPGKLKYSFFCNSGTESVEAALKLAKAYQSPRGKFTFIATSGAFHGKSLGALSATAKSTFRKPFMPLLPGFRHVPFGNIEAMRTALNECKKTGDDVAAVILEPIQGEGGVILPPPGYLTAVRKLCDEFGALMILDEVQTGMGRTGKMFACEHENVQPDILCLAKALGGGVMPIGATIATEEVFSVLFDNPFLHTTTFGGNPLACAAALATINVLLEQNLPAQAEQKGDMLLDGFRQLAREYPDLVQEARGKGMLMAIEFVDNEIGYNFASEMFRQRVLVAGTLNNAKTIRIEPPLTLTIEQCELVIKAARKALAAMRVSVEEA

SEQ ID NO: 5 - DNA, 1362 bp, Pseudomonas putida KT2440
  source 1..1362: mol_type = genomic DNA
atgagcgtcaacaacccgcaaacccgtgaatggcaaaccctgagcggggagcatcacctcgcacctttcagtgactacaagcagctgaaggagaaggggccgcgcatcatcaccaaggcccagggtgtgcatttgtgggatagcgaggggcacaagatcctcgacggcatggccggtctatggtgcgtggcggtcggctacggacgtgaagagctggtgcaggcggcggaaaaacagatgcgcgagctgccgtactacaacctgttcttccagaccgctcacccgcctgcgctcgagctggccaaggcgatcaccgacgtggcgccgaaaggtatgacccatgtgttcttcaccggctccggctccgaaggcaacgacactgtgctgcgcatggtgcgtcactactgggcgctgaagggcaaaccgcacaagcagaccatcatcggccgcatcaacggttaccacggctccaccttcgccggtgcatgcctgggcggtatgagcggcatgcacgagcagggtggcctgccgatcccgggcatcgtgcacatccctcagccgtactggttcggcgagggaggcgacatgacccctgacgaattcggtgtctgggccgccgagcagttggagaagaagatcctcgaagtcggcgaagacaacgtcgcggccttcatcgccgagccgatccagggcgctggtggcgtgatcatcccgccggaaacctactggccgaaggtgaaggagatcctcgccaggtacgacatcctgttcgtcgccgacgaggtgatctgcggcttcggccgtaccggcgagtggttcggctcggactactacgacctcaagcccgacctgatgaccatcgcgaaaggcctgacctccggttacatccccatgggcggtgtgatcgtgcgtgacaccgtggccaaggtgatcagcgaaggcggcgacttcaaccacggtttcacctactccggccacccggtggcggccgcggtgggcctggaaaacctgcgcattctgcgtgacgagaaaattgtcgagaaggcgcgcacggaagcggcaccgtatttgcaaaagcgtttgcgcgagctgcaagaccatccactggtgggtgaagtgcgcggcctgggcatgctgggagcgatcgagctggtcaaggacaaggcaacccgcagccgttacgagggcaagggcgttggcatgatctgtcgcaccttctgcttcgagaacggcctgatcatgcgtgcggtgggtgacaccatgatcatcgcgccgccgctggtaatcagccatgcggagatcgacgaactggtggaaaaggcgcgcaagtgcctggacctgacccttgaggcgattcaataa

SEQ ID NO: 6 - DNA, 1383 bp, Pseudomonas putida KT2440
  source 1..1383: mol_type = genomic DNA
atgaacgcgcctttcgccccgcaacgccagacccgtgactaccaggcagccgatgccgcccaccacattcatgccttcctcgaccagaaggcgctgaacgccgaagggccgcgggtgatcgtcggtggcgaacgcctgcacctgtgggacagcgagggcaagcgttacctggatggcatgtccggcctgtggtgcacccagctcggttatggccgtcgtgacctgacggccgccgcggccacgcagatggatcagctggcctactacaacatgtttttccacaccacccacccggcggtgatcgaactgtccgagttgctgttcagcctgctgccggggcactacagccacgcgatctacaccaactccggctccgaggccaacgaggtactgatccgcaccgtgcgccgctactggcaggtggttggccagccaggcaagaaaatcatgatcggccgctggaacggctaccacggctcgaccctggcggccacggcgctgggtgggatgaagttcatgcacgacatgggcgggttgattccggatgtggcacacatcgacgaaccctactggtacgccgagggcggtgaactgactccggccgagttcggccgccgctgcgccctgcagctggaggaaaaaatcctcgaactgggtgccgagaacgttgccggcttcattgccgaacccttccagggggccggcggcatgatcttcccgccggaaagctactggccggaaatccagcgtatctgccgccagtacgacgtgctgctgtgcgccgatgaggtgatcggtggctttggccgcaccggcgaatggttcgcccatgaatacttcggcttcgagcccgacaccttgtcgattgccaagggcctgaccagcggctatgtgcccatgggcggcctggtgctgagcaagcgcattgccgaggcgttggtggagcgcggcggggtatttgcccacggcctgacctattccggccacccggtggcggcggcagtggccatcgccaacctgaaggcgctgcgtgacgaaggcatcgtgcgccaggtgaaggacgacacggggccgtacctgcagcgcatcctgcgggaagtgtttgccgaccacccattgatcggccaggtgcaaggggccgggctggtggcggcgctgcagttcgccgagcacaagccgacgcgcaagcgctttgccaacgagaacgacctggcctggcagtgccgcacctttggtttcgaggaaggggtgatcattcgctcgaccctgggccggatgatcatggccccggccttgatcgccaaccacagcgagctggatgagctggtggagaagacccggatagccgtagaccgcacggcgcggctggtcggcaagctgtaa

SEQ ID NO: 7 - DNA, 1362 bp, Aeromonas salmonicida subsp. salmonicida
  source 1..1362: mol_type = genomic DNA
atgcagcacacgacacgtgagtggcagcagctggatgccagccaccacctgcatccctttaccgattttcaggcgctgaaccagaagggcagccgcatcatcaccagggccgaaggcatctatctggaagactccgacgggcgtcgcattctggacggtatggcgggactctggtgcgtcaacatgggctacggtcgtcaggagctggtggaggctgccaccaaacagatgcagcaactgccctactacaaccttttcttccagaccgcacaccctcctgtgatcgagttggcgaccctgctggccgaggtgactccgtcccatctcaatcatgtcttcttcaccggttctggctccgagtgcaacgatacggtgctgcgcatggtccgccactactgggccagcaaggggcagccggacaagcaggtgatcatcagccgccacaacgcctatcacggctccaccgtggcgggtgccagtctgggtggcatgaagggcatgcacgcccagggcggcctgcccattcccggcatagtgcacatcgatcagccctatcacttcggtgaggggcagggaatgagtgcccacgagtttggtctggagcgtgcccgccagctggagcagaagatcctggagctgggggtggacaaggtggccgccttcatcggcgagcccatccagggcgccggcggcgtcatcattccgcccgacagctactggcccgagatccagcgcatctgtgacaagtacggcatcctgctcattgccgacgaggtgatctgcggctttggccgtaccggccactggttcgccagcgagggattcggcatcaagccggacctcatgtgcctggccaagggcatcacctcaggctatctgcccatgggggccgtgatggtgggggatcgcgttgccagggtgctggtggaggagggcggcgaattcaaccacggcttcacctattccggtcatccggtggcctgcgccgtcgccattgccaacattaagcttatgcaaagcgaaagcatagttaagcgaattcatgatactatcggcccctatttgcagcgccgctggcgcgaactggcagaccatccgctggtgggcgaaacccgtggcaaaggcctggtggccgcgctggaaatagtgcaggacaagcagaccaacagccgcttcccggctgggctgcaagccggcatgacctgccgggaattctgctttaacaatggcttggtgatgcgggcggtcggcgataccatgatcatatcgccccccttggtcatcaccgaggaacaggtggatgaattggtcaatctggccaggctcagtctggatctgacggctgcaaagctgaaagggtag

SEQ ID NO: 8 - DNA, 1380 bp, Escherichia coli K12 MG1655
  source 1..1380: mol_type = genomic DNA
ttgaacaggttaccttcgagcgcatcggctttagcgtgcagcgcccacgccctgaatctcattgagaagcgaacgctggatcatgaggagatgaaagcacttaaccgagaggtgattgaatacttcaaagagcatgtcaatccggggtttttagagtatcgcaaatctgttaccgccggcggggattacggagccgtagagtggcaagcgggaagtttaaatacgcttgtcgacacccagggccaggagtttatcgactgcctgggaggttttggaattttcaacgtggggcaccgtaatccagttgtggtttccgccgtacagaatcaacttgcgaaacaaccgctgcacagccaggagctgctcgatccgttacgggcgatgttggcgaaaacccttgctgcgctaacgcccggtaaactgaaatacagcttcttctgtaatagcggcaccgagtccgttgaagcagcgctgaagctggcgaaagcttaccagtcaccgcgcggcaagtttacttttattgccaccagcggcgcgttccacggtaaatcacttggcgcgctgtcggccacggcgaaatcgaccttccgcaaaccgtttatgccgttactgccgggcttccgtcatgtgccgtttggcaatatcgaagccatgcgcacggctcttaacgagtgcaaaaaaaccggtgatgatgtggctgcggtgatcctcgaaccgattcagggtgaaggtggcgtaattctgccgccgccgggctatctcaccgccgtacgtaagctatgcgatgagttcggcgcactgatgatcctcgatgaagtacaaacgggcatggggcgcacgggcaagatgttcgcctgcgagcatgagaacgtacagccggatatcctctgccttgccaaagcgctcggcggcggcgtgatgccgattggcgcgaccatcgccactgaagaggtgttttcagttctgttcgacaacccattcctgcataccaccacctttggcggcaacccgctggcctgtgcggcggcgctggcgaccatcaatgtgttgctggagcagaacttaccggctcaggctgagcaaaaaggcgatatgttgctggacggtttccgtcaactggcgcgggaatatcccgatctggtacaggaagcgcgtggtaaagggatgttgatggcgattgagtttgttgataacgaaatcggctataactttgccagcgagatgttccgccagcgcgtactggtggccggaacgctcaataacgccaaaacgatccgcattgaaccgccactgacactgaccattgaacagtgtgaactggtgatcaaagcggcgcgtaaggcgctggcggccatgcgagtaagtgtcgaagaagcgtaa

SEQ ID NO: 9 - DNA, 18 bp, synthetic construct
  source 1..18: mol_type = other DNA
ggatccgtgatggtgatg

SEQ ID NO: 10 - DNA, 20 bp, synthetic construct
  source 1..20: mol_type = other DNA
aagcttaattagctgagctt

SEQ ID NO: 11 - DNA, 33 bp, synthetic construct
  source 1..33: mol_type = other DNA
caccatcacggatccagcgtcaacaacccgcaa

SEQ ID NO: 12 - DNA, 34 bp, synthetic construct
  source 1..34: mol_type = other DNA
cagctaattaagcttttattgaatcgcctcaagg

SEQ ID NO: 13 - DNA, 31 bp, synthetic construct
  source 1..31: mol_type = other DNA
caccatcacggatccaacgcgcctttcgccc

SEQ ID NO: 14 - DNA, 33 bp, synthetic construct
  source 1..33: mol_type = other DNA
cagctaattaagcttttacagcttgccgaccag

SEQ ID NO: 15 - DNA, 32 bp, synthetic construct
  source 1..32: mol_type = other DNA
caccatcacggatcccagcacacgacacgtga

SEQ ID NO: 16 - DNA, 34 bp, synthetic construct
  source 1..34: mol_type = other DNA
cagctaattaagcttctaccctttcagctttgca

SEQ ID NO: 17 - DNA, 33 bp, synthetic construct
  source 1..33: mol_type = other DNA
caccatcacggatccaacaggttaccttcgagc

SEQ ID NO: 18 - DNA, 34 bp, synthetic construct
  source 1..34: mol_type = other DNA
cagctaattaagcttttacgcttcttcgacactt

SEQ ID NO: 19 - protein, 474 aa, Escherichia coli K12 MG1655
MQHKLLINGELVSGEGEKQPVYNPATGDVLLEIAEASAEQVDAAVRAADAAFAEWGQTTPKVRAECLLKLADVIEENGQVFAELESRNCGKPLHSAFNDEIPAIVDVFRFFAGAARCLNGLAAGEYLEGHTSMIRRDPLGVVASIAPWNYPLMMAAWKLAPALAAGNCVVLKPSEITPLTALKLAELAKDIFPAGVINILFGRGKTVGDPLTGHPKVRMVSLTGSIATGEHIISHTASSIKRTHMELGGKAPVIVFDDADIEAVVEGVRTFGYYNAGQDCTAACRIYAQKGIYDTLVEKLGAAVATLKSGAPDDESTELGPLSSLAHLERVGKAVEEAKATGHIKVITGGEKRKGNGYYYAPTLLAGALQDDAIVQKEVFGPVVSVTPFDNEEQVVNWANDSQYGLASSVWTKDVGRAHRVSARLQYGCTWVNTHFMLVSEMPHGGQKLSGYGKDMSLYGLEDYTVVRHVMVKH

SEQ ID NO: 20 - protein, 487 aa, Pseudomonas putida CSV86
MRETKEQPIWYGKVFSSNWVEARGGVANVVDPSNGDILGITGVANGEDVDAAVNAAKRAQKEWAAIPFSERAAIVRKAAEKLKEREHEFADWNVRECGAIRPKGLWEAGIAYEQMHQAAGLAYLSNGTLFPSAVPGRMNLCQRVPVGVVGVIAPWNFPLFLAMRSVAPALALGNAVILKPDLQTAVTGGALIAEIFSDAGMPDGVLHVLPGGADVGESMVANSGINMISFTGSTQVGRLIGEKCGRMLKKVALELGGNNVHIVLPDADLDGAVSCAAWGTFLHQGQVCMAAGRHLVHRDVAQQYAEKLALRAKNLVVGDPNSDRVHLGPLINDKQVVRVHALVESAQSAGAKVLAGGTYQDRYYQATVIMDVKPEMEVFKSEIFGPVAPITVFDSIEEAIELANCSEYGLAASIHTRALATGLDIAKRLNTGMVHINDQPINCEPHVPFGGMGASGSGGRFGGPASIEEFTQSQWISMVEKPANYPF

SEQ ID NO: 21 - protein, 496 aa, Pseudomonas putida S12
MNSSLSAIDGLRLPHQMLIGGQWVSAQSGKTLNVYNPATGDILTEVPDGDVEDVNAAVESAAATLRSDTWRRMPPSARERILLRLADLLEVHGDELARLETLNNGKLLIYSKLMEVGASAQWLRYMAGWATKLTGSTLDLSLPLPPEVRSRASTQRVPVGVVAAIIPWNFPLLMAVWKIAPALACGNTVVLKPAEETPLTALRLAELAMEAGLPAGALNVVTGRGETAGDALVRHPKVAKVAFTGSTEVGRIIGSACGRSLKAVSLELGGKSPVIVLADCDPQEAAEGAAAAIFFNHGQVCTAGSRLYVHESIYEDVIQRLAVIGESIVVGSGLEQGVHMGPMVSKKHHENVLRHIRNGIEDGADLICGGTEAPCAQGFFVKPTIFANREKKDIRLLSQEVFGPVLVATPFSDIAEVVNEANRSVYGLGASIWTNDLSAALRINDELEAGTVWVNTHNMVDPNLPFGGFKDSGVGREHGAAAIEHYTTTRSLVIAY

SEQ ID NO: 22 - protein, 491 aa, Pseudomonas putida NCIMB 9866
MSQRLAAYENMSLQLIAGEWRVGKAGRDLDVLDPFTQEKLLQIPLANREDLDEAYRSARQAQVAWAACGPSERAQVMLNAVRIFDERRDEIIDWIIRESGSTRIKAQIEWGAARAITQESASLPSRVHGRILASDVPGKESRVYREPLGVIGIISPWNFPLHLTARSLAPALALGNACVIKPASDTPVTGGLLLAHIFEEAGLPKGVLSVVVGSGSEIGDAFVEHEVPGFISFTGSTQVGRNIGRIAAGGEHLKHVALELGGNSPFVVLADADLDQAVNAAVVGKFLHQGQICMAINRIIVEDSVYDEFVNRYAERVKSLPYGDPSKPETVVGPVINAKQLAGLQDKIATAKSEGARVMVEGEAQGNVLPPHVFADVTADMEIAREEIFGPLVGIQRARDEAHALELANSSEYGLSSAVFTSSLERGVKFARGIRAGMTHINDIPVNDEPNAPFGGEKNSGLGRFNGDWAIEEFTTDHWITVQHAPRRYPF

SEQ ID NO: 23 - DNA, 1425 bp, Escherichia coli K12 MG1655
  source 1..1425: mol_type = genomic DNA
atgcaacataagttactgattaacggagaactggttagcggcgaaggggaaaaacagcctgtctataatccggcaacgggggacgttttactggaaattgccgaggcatccgcagagcaggtcgatgctgctgtgcgcgcggcagatgcagcatttgccgaatgggggcaaaccacgccgaaagtgcgtgcggaatgtctgctgaaactggctgatgttatcgaagaaaatggtcaggtttttgccgaactggagtcccgtaattgtggcaaaccgctgcatagtgcgttcaatgatgaaatcccggcgattgtcgatgtttttcgctttttcgcgggtgcggcgcgctgtctgaatggtctggcggcaggtgaatatcttgaaggtcatacttcgatgatccgtcgcgatccgttgggggtcgtggcttctatcgcaccgtggaattatccgctgatgatggccgcgtggaaacttgctccggcgctggcggcagggaactgcgtagtgcttaaaccatcagaaattaccccgctgaccgcgttgaagttggcagagctggcgaaagatatcttcccggcaggcgtgattaacatactgtttggcagaggcaaaacggtgggtgatccgctgaccggtcatcccaaagtgcggatggtgtcgctgacgggctctatcgccaccggcgagcacatcatcagccataccgcgtcgtccattaagcgtactcatatggaacttggtggcaaagcgccagtgattgtttttgatgatgcggatattgaagcagtggtcgaaggtgtacgtacatttggctattacaatgctggacaggattgtactgcggcttgtcggatctacgcgcaaaaaggcatttacgatacgctggtggaaaaactgggtgctgcggtggcaacgttaaaatctggtgcgccagatgacgagtctacggagcttggacctttaagctcgctggcgcatctcgaacgcgtcggcaaggcagtagaagaggcgaaagcgacagggcacatcaaagtgatcactggcggtgaaaagcgcaagggtaatggctattactatgcgccgacgctgctggctggcgcattacaggacgatgccatcgtgcaaaaagaggtatttggtccagtagtgagtgttacgcccttcgacaacgaagaacaggtggtgaactgggcgaatgacagccagtacggacttgcatcttcggtatggacgaaagatgtgggcagggcgcatcgcgtcagcgcacggctgcaatatggttgtacctgggtcaatacccatttcatgctggtaagtgaaatgccgcacggtgggcagaaactttctggttacggcaaggatatgtcactttatgggctggaggattacaccgtcgtccgccacgtcatggttaaacattaa

SEQ ID NO: 24 - DNA, 1464 bp, Pseudomonas putida CSV86
  source 1..1464: mol_type = genomic DNA
atgcgtgagaccaaggagcaaccgatctggtatggcaaggtgtttagcagcaactgggtggaggcgcgtggcggcgtggcgaatgtggttgatccgagcaacggtgacatcctgggtattaccggcgtggcgaacggtgaagatgtggatgcggcggttaacgcggcgaagcgtgcgcagaaagaatgggcggcgatcccgttcagcgagcgtgcggcgattgttcgtaaggcggcggaaaagctgaaagagcgtgaacacgagtttgcggattggaacgtgcgtgagtgcggtgcgatccgtccgaaaggcctgtgggaagcgggtattgcgtatgagcagatgcaccaagcggcgggcctggcgtatctgagcaacggtaccctgttcccgagcgcggttccgggtcgtatgaacctgtgccagcgtgtgccggttggtgtggttggcgtgatcgcgccgtggaacttcccgctgtttctggcgatgcgtagcgtggcgccggcgctggcgctgggtaacgcggttattctgaagccggatctgcaaaccgcggtgaccggtggcgcgctgattgcggaaattttcagcgatgcgggtatgccggatggtgtgctgcacgttctgccgggtggcgcggatgtgggtgaaagcatggttgcgaacagcggtatcaacatgattagctttaccggcagcacccaagttggtcgtctgatcggcgaaaaatgcggtcgtatgctgaagaaagtggcgctggagctgggtggcaacaacgtgcacattgttctgccggacgcggatctggatggtgcggttagctgcgcggcgtggggtaccttcctgcatcaaggtcaagtgtgcatggcggcgggtcgtcacctggtgcaccgtgatgttgcgcagcaatacgcggaaaagctggcgctgcgtgcgaaaaacctggtggttggtgatccgaacagcgaccgtgttcacctgggcccgctgatcaacgacaagcaggtggttcgtgtgcatgcgctggttgagagcgcgcaaagcgcgggtgcgaaagttctggcgggtggcacctaccaggatcgttactatcaagcgaccgtgattatggacgttaagccggaaatggaagtgttcaaaagcgaaatctttggtccggtggcgccgattaccgtttttgacagcatcgaggaagcgattgaactggcgaactgcagcgagtatggcctggcggcgagcattcatacccgtgcgctggcgaccggtctggatattgcgaagcgtctgaacaccggcatggttcacatcaacgaccagccgattaactgcgaaccgcatgttccgtttggtggcatgggtgcgagcggtagcggtggccgttttggtggcccggcgagcatcgaggaatttacccagagccagtggattagcatggtggagaaaccggcgaactacccgttttaa

SEQ ID NO: 25 - DNA, 1491 bp, Pseudomonas putida S12
  source 1..1491: mol_type = genomic DNA
atgaacagcagcctgagcgcgattgatggtctgcgtctgccgcaccagatgctgattggtggccagtgggttagcgcgcaaagcggcaagaccctgaacgtttacaacccggcgaccggcgacatcctgaccgaagtgccggacggtgatgtggaggatgttaacgcggcggttgaaagcgcggcggcgaccctgcgtagcgatacctggcgtcgtatgccgccaagcgcgcgtgaacgtatcctgctgcgtctggcggacctgctggaagtgcacggcgatgaactggcgcgtctggagaccctgaacaacggcaagctgctgatttacagcaaactgatggaagttggtgcgagcgcgcagtggctgcgttatatggcgggctgggcgaccaaactgaccggtagcaccctggacctgagcctgccgctgccgccggaagtgcgtagccgtgcgagcacccaacgtgtgccggttggtgtggttgcggcgatcattccgtggaacttcccgctgctgatggcggtttggaagattgcgccggcgctggcgtgcggtaacaccgtggttctgaaaccggcggaggaaaccccgctgaccgcgctgcgtctggcggagctggcgatggaagcgggtctgccggcgggtgcgctgaacgtggttaccggtcgtggcgagaccgcgggtgatgcgctggtgcgtcacccgaaggtggcgaaagttgcgtttaccggcagcaccgaagtgggtcgtatcattggtagcgcgtgcggtcgtagcctgaaggcggttagcctggagctgggtggcaaaagcccggtgatcgttctggcggactgcgacccgcaggaagcggcggagggtgcggcggcggcgattttctttaaccatggtcaagtgtgcaccgcgggtagccgtctgtacgttcacgagagcatctatgaagatgtgattcagcgtctggcggttatcggcgagagcattgtggttggtagcggcctggaacaaggcgtgcacatgggtccgatggttagcaagaaacaccacgagaacgttctgcgtcacatccgtaacggcattgaagacggtgcggatctgatctgcggtggcaccgaggcgccgtgcgcgcagggtttctttgtgaagccgaccatcttcgcgaaccgtgagaagaaagacattcgtctgctgagccaagaagttttcggcccggtgctggttgcgaccccgtttagcgatattgcggaagtggttaacgaagcgaaccgtagcgtgtatggtctgggcgcgagcatttggaccaacgacctgagcgcggcgctgcgtattaacgatgagctggaagcgggtaccgtgtgggttaacacccacaacatggtggacccgaacctgccgttcggtggctttaaagatagcggtgttggtcgtgagcatggtgcggcggcgatcgaacactacaccaccacccgtagcctggttattgcgtattaa

SEQ ID NO: 26 - DNA, 1476 bp, Pseudomonas putida NCIMB 9866
  source 1..1476: mol_type = genomic DNA
atgagccagcgtctggcggcgtacgagaacatgagcctgcaactgattgcgggtgaatggcgtgtgggcaaggcgggtcgtgacctggatgttctggacccgttcacccaggagaaactgctgcaaattccgctggcgaaccgtgaggacctggatgaagcgtatcgtagcgcgcgtcaggcgcaagttgcgtgggcggcgtgcggtccgagcgagcgtgcgcaggttatgctgaacgcggtgcgtatctttgatgagcgtcgtgacgaaatcattgattggatcattcgtgaaagcggcagcacccgtatcaaagcgcagattgagtggggtgcggcgcgtgcgatcacccaagaaagcgcgagcctgccgagccgtgttcatggtcgtattctggcgagcgatgttccgggcaaagagagccgtgtgtaccgtgaaccgctgggtgttatcggcatcattagcccgtggaacttcccgctgcacctgaccgcgcgtagcctggcgccggcgctggcgctgggcaacgcgtgcgtgattaaaccggcgagcgacaccccggttaccggtggcctgctgctggcgcacattttcgaggaagcgggtctgccgaaaggcgtgctgagcgtggttgtgggtagcggcagcgaaatcggtgatgcgtttgttgagcacgaagtgccgggtttcattagctttaccggcagcacccaagtgggtcgtaacattggtcgtattgcggcgggtggcgagcacctgaagcacgttgcgctggaactgggtggcaacagcccgttcgttgtgctggcggacgcggatctggaccaagcggtgaacgcggcggttgtgggtaaatttctgcaccagggccaaatctgcatggcgattaaccgtatcattgttgaggacagcgtgtacgatgaatttgtgaaccgttatgcggagcgtgttaagagcctgccgtatggtgacccgagcaaaccggaaaccgttgtgggcccggttatcaacgcgaagcagctggcgggtctgcaagataagattgcgaccgcgaaaagcgagggtgcgcgtgttatggtggaaggcgaggcgcagggtaacgtgctgccgccgcacgtttttgcggatgtgaccgcggatatggaaatcgcgcgtgaggaaatttttggtccgctggttggcattcagcgtgcgcgtgatgaggcgcatgcgctggaactggcgaacagcagcgagtacggcctgagcagcgcggtgttcaccagcagcctggaacgtggtgttaagtttgcgcgtggtattcgtgcgggcatgacccacatcaacgacattccggtgaacgatgagccgaacgcgccgttcggtggtgagaagaacagcggtctgggccgtttcaacggtgactgggcgatcgaggaatttaccaccgatcactggattaccgttcagcacgcgccgcgtcgttatccgttttaa

SEQ ID NO: 27 - DNA, 36 bp, synthetic construct
  source 1..36: mol_type = other DNA
caccatcacggatcccaacataagttactgattaac

SEQ ID NO: 28 - DNA, 36 bp, synthetic construct
  source 1..36: mol_type = other DNA
cagctaattaagcttttaatgtttaaccatgacgtg

SEQ ID NO: 29 - DNA, 34 bp, synthetic construct
  source 1..34: mol_type = other DNA
caccatcacggatcccgtgagaccaaggagcaac

SEQ ID NO: 30 - DNA, 35 bp, synthetic construct
  source 1..35: mol_type = other DNA
cagctaattaagcttttaaaacgggtagttcgccg

SEQ ID NO: 31 - DNA, 33 bp, synthetic construct
  source 1..33: mol_type = other DNA
caccatcacggatccaacagcagcctgagcgcg

SEQ ID NO: 32 - DNA, 37 bp, synthetic construct
  source 1..37: mol_type = other DNA
cagctaattaagcttttaatacgcaataaccaggcta

SEQ ID NO: 33 - DNA, 32 bp, synthetic construct
  source 1..32: mol_type = other DNA
caccatcacggatccagccagcgtctggcggc

SEQ ID NO: 34 - DNA, 35 bp, synthetic construct
  source 1..35: mol_type = other DNA
cagctaattaagcttttaaaacggataacgacgcg

SEQ ID NO: 35 - protein, 474 aa, Citrobacter koseri ATCC BAA-895
MPHQLLINGELVSGEGEKQPVYNPATGEVILEIAEASPAQVDAAVRAADRAFAEWGQTTPKARAELLLTLADVIEENAQTFAELESQNCGKPLHCALNDEIPAIVDVFRFFAGAARCLNGLAAGEYLEGHTSMIRRDPVGVVASIAPWNYPLMMAAWKLAPALAAGNCVVIKPSEITPLTALKLAEFAKDIFPPGVLNVLFGRGKTVGDPLTGHEKVRMVSLTGSIATGEHIIQHTAPSIKRTHMELGGKAPVIVFDDADLDAVVEGVRTFGFYNAGQDCTAACRIYAQKGIYDALVEKLGAAVASLKTGSPNDESTELGPLSSQAHLERVTKAVEEAKALGHINVVTGGQKLDGAGYYFAPTLLAGAKQEDAIVQREVFGPVVSMTVFDDEEQVLAWANDTQYGLASSVWTKDVGRAHRLSARLQYGCTWVNTHFMLVSEMPHGGQKRSGYGKDMSLYGLEDYTVIRHIMVKH

SEQ ID NO: 36 - protein, 474 aa, Salmonella enterica subsp. enterica serovar Choleraesuis str. SC-B67
MQYQLLINGVLVDGEGERQSVYNPATGEVILEIAEASPAQVDAAVLAADSAFAEWGQTTPKARAECLLKLADSIEQNALEFARLESQNCGKPLHCVINDEIPAIVDVFRFFAGAARCLSGLAAGEYLEGHTSMIRRDPIGVVASIAPWNYPLMMAAWKLAPALAAGNCVVIKPSEITPLTALKLAALAKDIFPPGVLNVLFGRGQTVGDVLTGHEKVRMVSLTGSIATGEHILRHTAPAIKRTHMELGGKAPVIVFDDADLDAAAQGVRTFGFYNAGQDCTAACRIYAQRGIYDALVEKLGNAVSSLKMGAPEDESTELGPLSSLAHLKRVTAAVEEAKALSHIRVITGGSQTEGKGYYFAPTLLADAKQEDAIVQREVFGPVVSITVFDDEDQVLRWANDSRYGLASSVWTQDVGRAHRLSARLQYGCTWINTHFMLVSEMPHGGQKQSGYGKDMSLYGLEDYTLVRHIMVKH

SEQ ID NO: 37 - protein, 474 aa, Pectobacterium atrosepticum SCRI1043
MHDKLLIEGKLIAGNGEALAVFNPATGEQIAAIPQADLHQIDAAVLAAESAFAHWGQTTPKTRATLLLKIADAIEENAEVFAKLESLNCGKPYHAVLNDEVPAVADVFRFFAGAARCLSGSAAGEYLEGHTSMIRRDPVGVVASIAPWNYPLMMASWKLAPALAAGNCVVLKPAEQTPLTTFYLAHLLADILPAGVVNIVFGRGADIGDALTGHEKVNMVSLTGSIATGAHILAHTAASVKRTHMELGGKAPVIVFDDADIDQVVDGIRSFGFYNAGQDCTAACRLYVQRAVYDEVVEALGKAVATLKIGDPRDETTELGPLITEPQLERVMGFVERAKALPHITVVTGGERVKGTGFYFQPTVLAGAKQDDEIVQKEVFGPVISITSFDDEAQVIGWANASNYGLASSVWTRDIGRAHRLAACLQYGCTWVNTHFMLVSEMPHGGQKLSGYGKDMSMYGLEDYTIVRHIMIRH

SEQ ID NO: 38 - protein, 474 aa, Cronobacter sakazakii ATCC 29544
MQSQLLINGALVEGKGERLPVYNPATGEVLLEIAEASPEQVDAAVKSADAAFEQWRLTTPKERAEALLKLADVIEANAQTFAQLESKNCGKPLHCVAGDEIPAVADVFRFFAGAARCLNGLAAGEYLADHTSMIRRDPVGVVASIAPWNYPLMMAAWKLAPALAAGNCVVLKPSEITPLTALKLAELAKDIFPAGVLNVLFGRGQTVGDPLTSHEKVRMVSLTGSIATGEHIISRTASSIKRTHMELGGKAPVLVFDDADLDAVVEGIRTFGFYNAGQDCTAACRIYAQKGMYDTLVEKLGTAVGSLKTGAPEDETTELGPLSSQAHLERVSQAVEAAKALPHIRVVTGGAKIDGPGYYFQPTVLAGAKQEDAIVQREVFGPVISVTPFEDEAQALTYANDSQYGLASSVWTRDVGRAHRLSARLQYGCTWVNTHFMLVSEMPHGGQKLSGYGKDMSMYGLEDYTVVRHVMIKH

SEQ ID NO: 39 - protein, 474 aa, Pseudomonas putida KT2440
MQTQMLINGQLVAGQGPAWTVLNPALGTALAQINEATEAQVDSAVRAADQAFDSWSQTSPKERSQALLALADAIEAHGDELARLESQNCGKPLSAALNDEIPAIADVFRFFAGAARCLGGSAAGEYLPGHTSMIRRDPLGVVASIAPWNYPLMMLAWKIAPALAAGNTVVIKPSELTPLTALRLGELAQDLLPPGVLNILFGRGQTVGNPLITHPKVRMVSLTGSIPTGAHIISATADSVKRMHMELGGKAPVLVFDDADIDAAIDGIRTFGFYNAGQDCTAACRLYVQDGIYERFVERLGKAVASLKPGLQESEETELGPLISAQHRDKVAGLVQRAIAQPHIRLVTGGKPIAGDGFFFEPTVLADALQDDEIVRNEVFGPVVSVTRFTDEAQALEWANDSNYGLASSVWTRDTGRAHRLAARLQYGCTWVNTHFMLVSEMPHGGQKHSGYGKDMSMYGLEDYTCVRHVMIKH

SEQ ID NO: 40 - protein, 488 aa, Halioxenophilus aromaticivorans
MQQERREASIWSGKVFSSGWVEARGGVCDVTDPSNGDLLGVTGIANGEDVAAAAQTARRAQKGWAAIPFSERAEIVRKAAEKLKERENEFADWNVRECGAIRQKGLWEAGITYQQMHQAASLAFLPDGTSFPSAVAGRLNLCQRVPVGVVGVIAPWNFPLFLSMRSVAPALVLGNAVVLKPDPQTAITGGALIAEIFSEAGLPDGVLHVLPGGAEAGESMVASPEIDMISFTGSTQVGRLIGEKCGGMLKKVALELGGNNVHIVLPDADLDGAASCAAWGTFLHQGQVCMAAGRHLVHRDIAQEYAEKLALRARNLVVGDPKTDQVHLGPLINDKQVAHVHALVESAQKAGAKILAGGAYQDRYYQATVLMDVTPKMDVFKLETFGPVAPITVVDSVEEAIELANSSEYGLAASIHTKSLATGLEIARNLKTGMVHINDQPINCEPHVPFGGMGASGSSGRFGGLASIDEFTQSQWISMVEKPSIYPF

SEQ ID NO: 41 - protein, 487 aa, Sphingomonas sp. TF3
MNTPIKSNAWTGKVFSHGWSAGSGGVAEVIEPATGEVLGQIGIADVKDVDAAVASARSAQEAWAATPFDQRAAIIRTAAEVLKRRAAEFVQWNTRECGSIPPKGEYEVGITYEQLQQAAALAALPNGSLFPSSVPGRTNLWQRVPLGVVGVIAPWNFPLFLAMRSVAPALSLGNAVVLKPDLQSAVTGGVLIAEIFEEAGLPDGVLHVLPGGAETGEALVRHPDVAMISFTGSTAVGRSIAEICGRMLKKVALELGGNNVHIVLPDADLDGAASCAAWGSFLHQGQVCMAAGRHLVHRSVVDEYAAKLATRAGALHVGDPNAGPCHLGPLINDRQVARVHEVVTGSIEAGAEVLTGGVHEGRFYQPTVLKGVTPEMSAFKSEIFGPVAPITVFDTEDEAIALSNRSEYGLAASIHTASAARGLALAKRLKTGMVHINDQPINCEPQVPFGGMGASGSGGRFGGPASIDEFTQAQWISLVEKPVIYPF

SEQ ID NO: 42 - protein, 487 aa, Rhodococcus imtechensis
MRRLLDEPVWESRIFTGEWVRGSADDHPVVEPATGKQLSTIGMATADDVTRAADRAATAQADWAARPYTERAAVLRRAGTLFEQHADEIAEWVIREAGSIPTKAHIETHTAAEECYNAAALAAHPYGEVLRSEQPRLSFSRRIPVGTVGVIAPFNFPIILSIRAVAPALALGNAVVLKPDPRTAICGGAVLARIFEEAGLPAGLLSVLPGGADAGEAVVVHRTVRVIAFTGSTRAGRAVGELAGRHLKRSHLELGGNNALIVLDDVDLEKAVAVGAFGSFMHQGQICMAAGRHLVHESIAADYTALLAEHADRLPVGDPFTGDVALGPIIDAKQRDHIHTLVTASIDAGATLAAGGTYDDLFYRPTVLAQTPLTAAAFQDEVFGPVAPVASFSSIEEAVTIANSSEYGLSLSILTADAMKGLELAQRIPAGLVHVNDQTVGDEAVVPFGGVGSSGNGGRVGGISANLDAFTETQWVTAQSTMPAYPF

SEQ ID NO: 43 - protein, 486 aa, Rhodococcus ruber
MALLDESIWQGKIFTGDWTPGGGGEIKVVEPATGATLGSAGLADEGDLERAVDRAVAAQGDWAARPHTERAAVMRRAGVLWQQHADEIERWIMRESGSLRPKAQLETHVAAQECYEGAALPSHALGEILPSEAPRLSMSKRVPVGVVGVIAPFNFPLILAIRSVAPALALGNAVILKPDPRTAVCGGVALARIFEQAGLPAGVLSVLPAGADVGAALVDDPRVPVISFTGSTPAGRAVGAAASRNLKKVHPELGGNSAIVVLDDADLAATVSAGAAGSFLHQGQVCMTTGRHIVHESVYDEYVAQLAAKAEALPVGDPVTEQVALGPIIDQGQLEKIHALVTASVDAGARLVAGGTYEGLFYRPTVLADVPAGAPAYAQEVFGPVAPVVKFSTLDEAVALATDTDYGLSLGIFTRDVGKGLALADRIPTGIAHINDQTVGDEANIPFGGLGASGNGARFGGAANSIEAFTESRWITVSRDVPAYPF

SEQ ID NO: 44 - protein, 496 aa, Pseudomonas sp. LQ26
MNSSLPNIDGLLSPNQMLIGGEWVNARSDKTLSVYNPATGEVLTEVPDADAADVDAAVEGASATLQSGVWRHMAPVARERILLRLADLLEAHGDELARLETLNNGKLLIYSKLMEVGASAQWLRYMAGWATKLTGNTLDLSLPLPPQVRTKASTQRLPIGVVAAIIPWNFPLLMAVWKITPALACGNTVVLKPAEETPLTALRLAELALEAGLPAGALNVVTGRGESAGDALVSHPKIAKVAFTGSTEVGRVIGAACGRSLKAVSLELGGKSPVIVLPDCDPQKAAEGAAAAIFFNHGQVCAAGSRLYVHESIYEDVIQRLAVIGQSIVLGSGLDQAAQMGPMVSQKHHENVLRHIRNGIEDGVDLVCGGADSPALPGYFVQPTVFANRQKKDIRLLSQEVFGPVLVATPFSDIQEVISEANRSVYGLGASIWTNDLSAALRINDELEAGTVWVNTHNMVDPNLPFGGFKDSGVGREHGAAAIEHYTTPRCHHIQC

SEQ ID NO: 45 - protein, 500 aa, Burkholderia lata
MYREISMPLEVTGSSLRTSMFINGEWQQANSGKMIPVFDPSNGERIASVPDADVADIDRAVESASLTFRSTSWKSMPPAARERILLRLADLIEKHGEELAALETRNNGKLIAYSRMFEVGAGTQWLRYMAGWATKISGSTLDLSLPLPPTVRTSAFTRRIPVGVVGAIIPWNFPLLMAVWKIAPALACGNTVVLKPAEETPLTALRLAELAVEAGLPAGALNVVTGRGETAGAALVAHPKVSKVTFTGSTEVGRLIGATCGQNLKPASLELGGKSPVIVLNDCDPDVAARGAADAIFFNHGQVCTAGSRLYVHHDIYDDVLDRLSAIADTIVVGSGFDESAHMGPLVSLRHQQRVKSLIESGRADGAEQLCGAGATPENGYYVRPTVFANHDNRPMRLLTEEVFGPVLVAMPFTDLAEVVDEANDSAYGLGASVWTNNLSASLALTEAIEAGTVWVNTHNMVDPNLPFGGFKDSGIGREHGASAIENYTTTKSVCIAYQG

SEQ ID NO: 46 - protein, 492 aa, Paraburkholderia sp. 5N
MTEQKTTAKLPTAMFINGEKTLSAAGKTFPIYNPATGQELSQIPDASETDIDHAVKTSKAAFESDTWRRMPPATRERLLLKLADLVEQHTDELATLETLNQGKLIVFSKMLEVTGSVQWLRYMAGWATKIEGTTFDLSVPFPPGTRYNASTKRVPAGVVAAIVPWNFPLLVAVWKIAPALACGCTVVLKPAEETPLTAIRLAELAHEAGFPPGVFNVVTGRGETAGAALVKHPLINKVTFTGSTEVGRIIGRQCADDLKRASLELGGKSPVIVLDDCDPKKAIEGAAGAIFFNHGQVCTAGSRLYVARSIYDEVVQGIAAVADGIALGSGFDAATQMGPMVSARHRDKVMGMIAQGRQEGGEILSRDAAVDAVGFFVRPTVIANRACKPLSVVREEVFGPVLVAMPYDDIDEVLAQANASEYGLGASVWTNQLDKALRLVDGIEAGTVWVNTHNMVDPAMPFGGFKASGIGREHGKAIVDSYTESKSVCIAY

SEQ ID NO: 47 - DNA, 1425 bp, Citrobacter koseri ATCC BAA-895
  source 1..1425: mol_type = genomic DNA
atgccgcatcagctgttgattaacggggaactggtatcaggggaaggagaaaagcaaccggtctataatccggcaaccggcgaagttatcctggaaattgcggaagcgagccccgcacaagtcgatgcagcggttcgtgcggcagatcgtgcgtttgccgaatggggccaaaccacaccgaaggcgcgtgcggaactcctccttacactggccgacgtcatcgaggaaaatgcccaaacgttcgccgaactcgagtcacagaattgcggtaaacccctgcattgcgccttgaatgacgaaattccagcgattgtggatgtgttccgcttctttgctggtgctgcccggtgtctgaatggtctggccgcaggggaatatctcgaaggtcatacatccatgattcgccgtgacccagtgggagtggttgcgtcgattgccccgtggaactatccgctgatgatggcggcttggaaactggctccagcgttagcagccggcaactgcgtcgttattaagccgtcagaaatcacgccactgacggcgctgaaactggcggagttcgccaaagacatctttcctcctggcgttttaaacgtgctgtttggtcgtggcaaaaccgtaggagatccgcttaccggccacgagaaagtgcgtatggtttcgcttacgggcagtatcgccactggcgaacacatcattcagcataccgccccgagcatcaaacgcacacatatggaactgggcggtaaagctcctgtcattgtgttcgatgatgcagatctggatgccgttgtagaaggtgtacggaccttcggcttttacaacgctggccaagattgcacggctgcatgtcgcatttacgcacagaaaggcatttatgacgccctggtagagaagctgggtgcggcggttgcaagcttgaaaaccggctctccgaacgatgagtccaccgagttgggtccgttaagcagtcaagcgcatctggagcgcgtgactaaagctgttgaagaagccaaagcgcttggccacatcaacgtcgtgactggtgggcagaaattggatggggcaggatactactttgcaccgactctgttagcgggcgcgaaacaggaggatgcgattgttcagcgcgaagtgtttggtcctgtggtcagtatgacggtctttgacgacgaggaacaggtgctggcttgggccaatgatacgcagtatgggttggcaagctctgtttggaccaaagacgtgggtcgcgctcatcgtctgtctgcgcgcttacagtacggctgtacctgggtaaacacccactttatgctggtgtccgaaatgccccatggaggtcagaaacgctcgggttatggtaaggacatgagcttatatggcctggaagattacaccgtgattcgccacatcatggtcaaacactaa

SEQ ID NO: 48 - DNA, 1425 bp, Salmonella enterica subsp. enterica serovar Choleraesuis str. SC-B67
  source 1..1425: mol_type = genomic DNA
atgcagtatcaactgctgattaatggcgtcttagtggacggcgaaggtgaacgccagtcagtctacaaccctgccaccggtgaggtaatcctggaaattgcggaagccagtccggcacaggtagatgcggctgttcttgcggcggatagtgcatttgcggaatggggtcaaaccaccccgaaagctcgtgcagaatgcctgctgaaactggcggatagcattgagcagaacgcactggaattcgcccgtttagagtcccaaaactgcggtaaacccttgcattgcgtgatcaacgacgaaattccggccatcgtagacgtctttcggttctttgcaggggctgcacgctgtctttctggtctggcggcgggcgaatacctggaaggccacacgagcatgattcgccgtgacccgattggagtcgtcgcgagtatcgcgccttggaactacccgctgatgatggccgcttggaaattggcaccagcactcgcggccggcaattgcgtagttatcaaaccgagcgaaattaccccgctgacggcgcttaaacttgccgcattggcaaaggatattttcccgccgggcgtcctgaatgtcttatttggccgtggtcagactgttggtgatgtgctgacaggtcacgaaaaggttcgcatggtgagtctgacaggttctattgccacaggagagcatattctgcgccatactgccccagcgatcaagcgtacgcacatggaactgggtggtaaagctcccgtgattgtgtttgacgatgctgatctggatgccgccgctcaaggcgttcgcacctttggcttttacaacgcgggacaagactgtacggctgcttgtcggatctatgcgcaacgtggcatctatgatgccctggtagaaaagttgggcaatgcggtgtcatccctgaaaatgggcgcgccggaagatgagtctacggaactcggaccactgtcctcattagcacatctcaaacgcgtgaccgcggccgttgaagaggccaaagctctgtcgcacattcgtgtaatcactggcgggagccagaccgaaggtaaagggtactatttcgccccaaccctcttagccgatgcgaaacaagaggatgcgattgtgcagcgtgaggtgtttggtcctgtcgtgtcgatcacggttttcgacgacgaggatcaggtgttacgttgggcgaatgattcgcgctatgggttggcgtccagcgtttggacccaggatgtgggtcgcgcacatcgcctgtcggcacgcttgcagtatgggtgtacctggatcaacacccacttcatgctggttagcgaaatgccgcatggcggccagaaacagtctggctatggcaaagacatgagcctttatgggctcgaagattacactctggttcgccacattatggtgaaacattaa

SEQ ID NO: 49 - DNA, 1425 bp, Pectobacterium atrosepticum SCRI1043
  source 1..1425: mol_type = genomic DNA
atgcacgacaaactgctgattgagggtaaactgatcgccggaaatggtgaagctctggcggtgtttaaccctgcgactggcgagcagattgcggcaattccacaggcagatcttcatcagattgatgcagccgtcttagcggctgaaagcgcctttgcccattggggccagacaaccccgaaaactcgcgctacgctgttacttaaaatcgcggacgccattgaggaaaatgccgaagtgtttgcgaaactggaatcgcttaactgcggcaaaccgtaccatgcagtgttgaacgacgaagttccagccgttgcggatgtgttccgcttctttgcgggagctgcccgttgtctgagcggctcagcggccggtgaatacttggaggggcatacctcgatgatccggcgtgatccggtgggagtagtggcgagcattgcgccgtggaactatccgctgatgatggctagctggaaactggcacccgccttagccgcgggtaattgcgtcgtgttgaaacccgcggaacaaacgccactcaccaccttttacctggcacatctgttagcggatattctgcctgctggtgtcgtaaacatcgttttcggtcgtggggctgatattggcgatgcattaaccgggcatgaaaaggtgaacatggtaagtctgaccgggtctattgccaccggcgcacatatcctggcacacacggccgcgtccgtaaaacgtacacacatggaactcggtggcaaagctccagtgattgtctttgatgatgccgacattgaccaagttgtcgacggcatccgctctttcggcttctataatgccggtcaagattgcaccgcggcatgtcgcctctacgtgcaacgcgcagtatatgatgaggtcgttgaagcgttgggtaaagcggttgcgaccctcaaaattggggatcctcgtgacgagacaacagaactgggtccgctgatcactgaaccgcaactggaacgcgtaatgggatttgtcgagcgtgctaaagccctgccgcacatcacggtcgtgactggaggtgaacgtgtgaagggcacggggttttacttccagccgactgttctggccggtgcgaaacaggatgacgaaatcgtgcagaaggaggttttcggcccggtgattagcattacgtcgtttgatgacgaagctcaggtcatcggttgggcaaatgcgagtaactatggcttggcgtcaagtgtgtggacccgcgatattggtcgcgcacatcggcttgcagcgtgcttacagtacggttgtacgtgggttaatacccactttatgctggtttccgaaatgccgcatggcggccagaagctgtctggctatggcaaagacatgtccatgtatggcctggaagattataccattgttcgccacatcatgatccgccactga

SEQ ID NO: 50 - DNA, 1425 bp, Cronobacter sakazakii ATCC 29544
  source 1..1425: mol_type = genomic DNA
atgcagagtcaattactgattaacggcgcgctggtggaaggcaagggcgagcgcctgccagtctataaccccgcgacgggcgaggtgctgctggagattgccgaagccagcccggaacaggtggatgcggcggtgaagagtgccgacgcggcgtttgaacagtggcgtctcaccacgcctaaagagcgcgccgaggcgctgctcaagcttgcagatgtgattgaggccaacgcgcagacctttgcgcagcttgaatctaaaaactgcggcaagccgctgcactgcgtggcgggtgacgaaatcccggcggtggcggatgtgttccgcttctttgccggcgccgcgcgctgcttaaacgggcttgccgccggggaatacctggcggatcacacctcgatgatccgccgtgacccggtgggcgtggtcgcgtccatcgcgccgtggaactacccgctgatgatggccgcctggaagctggcccccgcgctggcggcgggcaactgcgtggtgcttaagccctctgaaattacgccgctgaccgcgcttaagctcgcggagcttgccaaagatatcttcccggcgggtgtgcttaatgtgctgtttggccgtggccagacggtgggcgacccgctcaccagccatgagaaagtgcgcatggtgtcgctcaccggctctatcgccaccggcgagcacatcatcagccgcaccgcgtcgtccatcaagcgcacccatatggagcttggcggcaaagcgccggtgctggtgtttgacgacgccgatctcgacgccgtcgtcgaaggcatccgcacctttgggttctataacgcgggccaggactgtacggcggcgtgccgcatctacgcccaaaaagggatgtacgacacgctcgttgaaaaactcggcaccgcagtcggcagcctgaaaacaggcgcgccggaggatgaaaccaccgaactcgggccgctcagttcacaagcgcacctggagcgcgtgagccaggcggtggaggcggcgaaagcgctgccgcatattcgcgtggtgactggcggcgcgaaaatcgacgggccgggctattactttcagccgaccgttctcgccggcgcgaagcaggaggacgctatcgtgcagcgcgaggtgtttggcccggttatcagcgtgacgccgtttgaggatgaagcccaggcgctgacctacgccaacgattcgcaatatggcctggcgtcatccgtatggacccgcgacgtgggccgcgcgcaccgcctcagcgcccgcctgcaatatggctgcacctgggtgaatacgcacttcatgctggtgagcgaaatgccccacggcggccagaaactctccggctacggaaaggatatgtcgatgtacgggcttgaggattacaccgtcgtgcggcatgtaatgataaaacactag

SEQ ID NO: 51 - DNA, 1425 bp, Pseudomonas putida KT2440
  source 1..1425: mol_type = genomic DNA
atgcaaacgcagatgctgatcaatggccagctggtcgctggccaaggcccggcctggaccgtgctcaacccggcgctgggcactgccctggcgcagatcaacgaagccaccgaggcgcaggtggacagtgccgtgcgcgctgccgaccaggccttcgacagctggtcgcaaaccagccctaaagaacgttcgcaggccttgctggcgctggccgatgccatcgaagcccatggcgatgaactggcccggctggaatcacagaactgcggcaagcccctgagcgctgcactcaacgacgagatcccggcgattgccgacgtgttccgtttctttgccggtgcggcgcgctgcctgggcggctcggcggcaggcgagtacctgccgggccacacctcgatgatccgccgcgacccgttgggcgtggtggcttccatcgcgccgtggaactacccgctgatgatgctggcctggaagatcgccccagccctggctgccggcaacaccgtggtgataaagccgtccgagctgacgccgctgacggccctgcgcctgggcgagctggcccaggacttgctgccgccgggggtgctgaacattctcttcggccgcggccagacggtcggcaacccgttgataacccaccccaaggtgcgcatggtgtcgctgaccggctcgatccccaccggcgcgcacatcatcagcgccaccgccgacagcgtgaaacgcatgcacatggagctgggcggcaaggcgccggtgctggtgttcgatgacgctgacatcgatgccgccatcgacggcatccgcaccttcggcttctacaacgccggccaggactgcaccgcagcctgccgcctgtatgtgcaggacgggatctacgagcgctttgtcgaacgcctgggtaaagccgtagccagcctcaagccgggcctgcaggagtctgaagaaaccgaactggggccactgatcagcgcccagcaccgcgacaaggtcgccgggctggtgcagcgggccatcgcccagccgcacattcgtctggtaaccggtggcaagccaatagcgggcgatggctttttcttcgagcctaccgtgctggccgacgccctgcaggacgacgagatcgtgcgcaacgaagtgtttggcccggtggtttcggtcacccgcttcaccgatgaagcgcaggcactggaatgggccaacgactccaactacggcctggcctcatcggtatggacccgcgacaccggccgcgcccaccgcctggcggcgcgcttgcagtatggctgcacctgggtgaatacccacttcatgctggtcagcgaaatgccccatggcgggcagaagcattcggggtatggcaaggacatgtcgatgtatgggctggaggactacacctgtgtgcggcatgtgatgatcaagcattga

SEQ ID NO: 52 - DNA, 1467 bp, Halioxenophilus aromaticivorans
  source 1..1467: mol_type = genomic DNA
atgcaacaggagcgtcgcgaagcatcgatttggagtggtaaagtgtttagctccggttgggtggaggcacgtggcggagtttgcgacgtgaccgatccaagcaatggcgatctgcttggtgtcacagggattgccaatggtgaggacgtcgcagcggcagcacagacagcccgtcgcgctcagaaaggctgggctgcgatcccgttctccgaacgtgctgaaatcgtgcgtaaagcagccgagaagctcaaagaacgcgagaacgaattcgccgattggaatgtccgcgaatgtggtgccattcgccagaaagggctgtgggaagctggcatcacctatcagcagatgcatcaagcggctagtctggcgtttctgccggatggcacctcctttccgtcagcggttgccggtcgcttaaacctgtgtcaacgtgtgcctgtaggagtggtcggagtgattgctccgtggaactttccgctgttccttagcatgcgttctgtggcgccagcgttggttctcgggaatgccgtagtactgaaaccggatccacagacggccattacgggcggagccttgatcgcggagatcttctctgaagcaggcttaccggatggtgtcttacacgttctgccgggtggtgcagaagcgggcgaaagcatggttgcttcgccagagatcgacatgatctcatttactggcagcactcaggtcggccgcctgatcggcgagaaatgcggcggcatgctgaagaaagtggctttagaacttggtgggaataacgtgcacattgtgcttcctgacgcagatttggatggcgcggcgtcttgtgcggcctggggtacgttcctgcatcaggggcaagtatgcatggcggcaggccgtcacctggtgcatcgcgacattgcacaggagtatgcggagaagctggccttacgggctcgcaatctggttgttggggatccgaaaacggatcaagtccatctcggtcctctgatcaacgacaaacaagtagcgcatgttcatgcgctggtagaatcggcccagaaagcgggagcaaagattctggccggcggtgcgtaccaggatcgctactatcaggctaccgttctcatggatgttacgccgaaaatggacgtgttcaaactggaaacatttggccccgtggcccctattaccgtcgtagattcggtcgaagaagcgatcgaattggcgaacagttcggaatatggcctggcggcgagcatccacaccaaatctttggccactggtctggaaattgcccgcaatctgaaaaccggcatggtgcacattaacgatcaaccgattaactgcgaaccccatgttccgtttggcgggatgggtgccagtggtagttccgggcggttcggtggcctggcatcaattgacgaatttacccagagccaatggatttcaatggtggaaaagcccagcatttacccgttttga

SEQ ID NO: 53 - DNA, 1464 bp, Sphingomonas sp. TF3
  source 1..1464: mol_type = genomic DNA
atgaacaccccgatcaagtcaaacgcttggactggtaaagtgttttcccacggctggtctgcaggcagcggtggggtagccgaagtgatcgagccggcaaccggagaagtactggggcagattgggattgcggatgtcaaagatgttgatgcggccgtcgctagcgctcgttcggcgcaggaagcgtgggctgctacccctttcgaccagcgtgccgccatcattcggacagctgcagaagtccttaaacgccgtgctgcggaatttgttcagtggaatacgcgcgaatgcggttccattccgccgaaaggggagtatgaggtggggattacctacgaacagctgcaacaggcggctgctcttgccgcgttgccaaacggatcgctgtttccctcatccgtgcctggacgtaccaatctgtggcagcgcgtgccactcggagtcgttggcgttatcgcaccttggaactttccgttgttcctcgcgatgcgtagcgtggcgcctgcattatcgttgggcaatgccgtggtgttaaaaccggatctccaatcagcagttacaggtggcgttctgattgcggaaattttcgaagaagccgggcttccggatggcgttttgcacgtgttacccggcggggccgaaacgggtgaagcgctggtgcgccatcccgacgtagcgatgatttcctttacgggtagtaccgcggttggccgtagcattgccgagatttgtggccgcatgctgaagaaagttgctctggagctgggtggcaataacgtgcacattgtcctgccggatgcggatctcgatggcgcagcgagttgtgcggcgtggggttcattcctgcatcaaggccaagtctgcatggccgcaggccgtcatcttgtgcatcgcagcgtcgtggacgagtatgcggcgaaactggcaacccgcgccggtgccttacatgtaggggacccaaatgccggtccttgtcacctgggtccgctgatcaacgatcgccaagtagcgcgcgttcatgaggtagttacgggatcgatcgaagcgggtgcagaagtgctgacgggcggtgtgcatgaaggccgcttttaccagccaactgtgctgaaaggcgtcacaccggaaatgtcggcgttcaaaagcgaaatcttcggcccggttgcaccgattactgtctttgatacggaagatgaggctattgccctgagtaaccgcagcgaatatggcttagcagcatctattcacaccgcgtctgcggcacgcggtctggccctggccaagcggttgaaaactggtatggtgcacatcaacgaccaaccgatcaattgcgaaccacaggtaccgtttggtggcatgggagcctctggcagtggcggtcgtttcggtggccccgccagcatcgacgaatttacccaggcacagtggatcagtctggtggagaaaccggtcatttacccgttttaa

SEQ ID NO: 54 - DNA, 1464 bp, Rhodococcus imtechensis
  source 1..1464: mol_type = genomic DNA
gtgcggcggttgctggacgaaccggtgtgggaatcacgaatcttcaccggcgaatgggtacgcggcagcgccgacgaccaccccgttgtcgagcccgcaaccggcaaacaactctcgaccatcggcatggccaccgcagacgatgtgacacgtgccgcggaccgagccgcgaccgcgcaagccgactgggccgcccgcccctacaccgaacgggcagcagtgctccgccgcgccggaaccctgttcgagcagcacgccgacgaaatcgccgaatgggtgatccgcgaggccggcagcatccccaccaaggcccacatcgaaacacacaccgccgccgaggagtgctacaacgctgcggcgcttgccgcacacccctacggtgaagtgctgcgctcggagcagccgcgcttgagcttctcccgccgcatcccggtgggcaccgtcggggtgatcgcccccttcaacttcccgatcatcctgtcgatccgtgccgtcgcgccggcgttggcgctcggtaacgccgtcgtcctcaagcccgacccccgcaccgccatctgtggcggtgcggtcctcgcccgcatcttcgaggaagccggccttcccgccggcctgctcagcgtgctgcccggcggcgccgacgccggggaagccgtcgtcgtccaccgcaccgttcgggtcatcgccttcaccggttcgacccgcgccgggcgtgccgtcggtgaactcgccggacggcacctcaaacgctcccacctcgaactcggtggcaacaacgccctgatcgtgctcgacgacgtcgacctcgagaaggccgtagccgtcggcgctttcggctccttcatgcaccagggccagatctgcatggcggcgggccgtcacctggtgcacgagagcatcgccgccgactacaccgcactcctcgctgaacacgccgaccggctgcccgtcggtgacccgttcaccggcgacgtcgccctcggcccgatcatcgatgccaaacaacgagatcacatccacaccctggtcaccgcgagcatcgatgcgggcgccaccctcgcggccggcggaacctacgacgatctcttctaccggcccaccgtgctcgcgcagaccccgctgaccgccgcggccttccaggacgaggttttcggcccggtagccccggtggcatcgttcagttcgatcgaggaagccgtgacgatcgccaacagctccgaatacgggctgtcgttgagcatcctgacagccgacgccatgaagggcctcgaactcgcacagcggatccccgccggcctggtgcacgtcaacgaccaaaccgtgggcgacgaggcagtagtcccgttcggcggcgtcggatcctcgggcaacggcgggcgggtcggcggcatcagcgccaacctcgacgccttcaccgaaacacagtgggtcaccgcgcaaagcacgatgcccgcttacccgttctga

SEQ ID NO: 55 - DNA, 1461 bp, Rhodococcus ruber
  source 1..1461: mol_type = genomic DNA
atggcccttctcgacgaatccatctggcagggaaaaatcttcaccggggactggacccccggcgggggcggtgagatcaaggtcgtcgaaccggcgaccggcgcgacgctcggcagcgccggcctcgccgacgagggggacctcgagcgcgcggtcgaccgtgccgtcgcggcccagggcgactgggcggcccgcccgcacaccgagcgtgccgcggtcatgcgccgggccggcgtcctgtggcagcagcacgccgacgagatcgagcgctggatcatgcgcgagtccggctccctgcgtcccaaggcgcagctcgagacgcacgtcgcggcgcaggagtgctacgagggtgcggccctgccctcccatgcgctcggcgagatcctgcccagcgaggcaccgcgtctgagcatgtcgaagcgggtccccgtcggggtcgtcggtgtcatcgcgccgttcaacttcccgttgatcctcgcgatccgttccgtcgcgccggcgctggccctcggcaacgccgtgatcctcaagcccgacccgcgtaccgcggtctgcggcggcgtggcgctcgcccgcatcttcgagcaggcgggcctgccggccggggtgctgtccgtgctgcccgccggcgccgacgtcggcgccgcgctcgtcgacgacccgcgggtgccggtgatctccttcaccggttccaccccggccggccgggccgtcggtgccgccgcctcccgcaacctcaagaaggtccaccccgaactcggcggcaactccgcgatcgtcgtgctcgacgacgccgacctcgccgccaccgtctcggccggtgccgccggatccttcctgcaccagggccaggtgtgcatgaccaccggccggcacatcgtgcacgagtccgtctacgacgagtacgtcgcccagctcgccgccaaggccgaggcactgcccgtcggcgaccccgtcaccgagcaggtcgcgctcgggccgatcatcgaccagggtcagctcgagaagattcatgccctggtcaccgcgtcggtcgatgccggcgcccggctcgtcgccggcggcacctacgagggcctgttctaccggcccaccgtcctcgccgacgtcccggccggtgcgcccgcctacgcccaagaggtgttcgggcccgtcgctccggtcgtgaagttctcgaccctcgacgaggcggtggcgctggccaccgacaccgactacgggctctcgctcggcatcttcacccgcgacgtcggcaagggtctcgcgctcgcggaccggatccccaccggcatcgcccacatcaacgaccagaccgtcggcgacgaggccaacatcccgttcggcggtctcggcgcctccggcaacggcgcccgcttcggcggtgccgccaacagcatcgaagcgttcaccgagtcgcgctggatcaccgtcagccgcgacgtgcccgcttaccccttctga

SEQ ID NO: 56 - DNA, 1491 bp, Pseudomonas sp. LQ26
  source 1..1491: mol_type = genomic DNA
atgaacagctcacttccgaacattgacggtctgcttagccctaaccagatgctgattggtggcgaatgggtaaatgcccgctcggacaaaaccttgtccgtgtataatccggcaactggtgaagtgctgaccgaggttccggatgcggatgcggcagacgtagacgcggccgtggaaggcgctagtgccaccctccagtctggtgtgtggcgtcatatggctccagtggcacgtgaacgcatcctgctgcgcttagcggatctgctggaagcgcatggggatgaactggctcgcttggaaaccctcaacaatgggaaacttctcatctattcgaaactgatggaagtgggcgcaagcgcccaatggctgcgctatatggcggggtgggcgaccaagctgacgggtaacactctggacctgtcattaccgctgccgccgcaagtgcgtaccaaagcctctacgcagcgtctgcccattggagttgtagcagccatcattccctggaactttccgctgttaatggccgtttggaaaatcaccccagcgttagcttgcggcaataccgtcgtgctgaaaccggcggaggaaaccccgctgacagcgctccggttggcggaacttgcgctggaagcaggcttgcctgctggtgcactgaacgtggtaactggacgcggtgaaagcgccggggatgcgttagtcagccatccgaaaattgccaaagtggcttttaccggaagtaccgaagttggccgggttattggggcggcatgtggtcgctctctgaaagcggtaagcctggaactgggcggcaaaagtccggtaatcgtccttcccgactgtgatccgcagaaagcggcagagggcgcagctgccgcgatcttcttcaaccacggtcaagtttgcgccgcaggatctcgtctgtatgtccatgagtcgatttacgaggatgtcatccaacgcctggctgtgattggccagtccatcgtcttggggtccggcctcgatcaagccgcccagatgggcccaatggtatcgcagaaacaccacgagaacgttttacgccatattcgcaatggcattgaagatggcgtggatctggtttgtggtggcgcggatagcccggcacttccaggttactttgtgcaacctacggtgtttgcgaatcgccagaagaaggacattcgcctgctcagtcaggaggttttcggtcccgttttagtcgctacaccgtttagcgatattcaggaggtgatctcggaagcaaatcgttcagtctatggcttgggcgcgagtatctggacgaatgatctgtcagccgccctgcgtatcaacgacgaactggaagccggaactgtctgggttaatacgcacaacatggtcgacccgaacttgccatttggcgggttcaaggattccggtgtgggtcgtgagcatggtgcggcggctattgaacactacacaacgcctcgttgccatcacattcagtgctga

SEQ ID NO: 57 - DNA, 1503 bp, Burkholderia lata
  source 1..1503: mol_type = genomic DNA
atgtatcgcgaaatttctatgccgctggaagtaaccggttcttctctgcgtaccagcatgttcatcaacggtgaatggcaacaggccaattccggcaagatgattccggtgtttgatccgtcaaacggtgagcgtatcgcctccgttccggatgcggacgtagcggacattgatcgcgccgttgagagtgcttcgctcactttccgcagtacctcgtggaaaagcatgcctccagcagcgcgcgaacgcattttactgcgtctggcagatctgatcgagaaacatggcgaagagctggccgcacttgaaacgcgcaacaacggcaagttgattgcgtatagtcggatgttcgaggttggcgctggtacccaatggctgcgctatatggcagggtgggcgactaagatttccggtagcaccctggatctctctctccctctgccgccaacagtgcgtactagtgcatttactcgccgcattcccgtgggtgtggtgggtgcgattatcccgtggaactttccgctgctgatggctgtctggaaaatcgccccagcgttagcgtgcggtaataccgtagttctgaaaccagccgaagaaaccccgctgactgccttacgtttagccgaattggcggttgaggccggattgcctgcgggcgcactgaatgtagtcacaggccgtggcgaaaccgcaggagcagcactggttgcccatccgaaagtcagcaaagtgacctttaccggcagcacagaagttggtcgtcttattggggcgacgtgtggtcagaaccttaaaccagcgagcttggaacttggagggaaatctccggtgattgtcctgaacgactgcgacccggatgtcgcagctcgtggtgctgcagatgctatcttcttcaatcatggccaggtgtgtactgcggggtcccgtctgtacgttcatcacgacatctacgatgatgtgcttgaccgcctgagcgcgattgccgatacgatcgttgtcggcagcggctttgacgaatcagcgcacatgggtccgctggtgtcgctccgtcatcagcaacgcgtcaaaagcttaatcgaatcaggccgcgctgatggagcagaacagctgtgtggtgctggcgccacgcccgaaaacgggtactatgttcgcccgaccgtgtttgcgaatcacgataatcggcccatgcggctgctgaccgaggaagtatttggccccgtgttggtagcaatgccgtttaccgatctggctgaagtggtggacgaagccaatgacagcgcgtatggcctcggcgcgagtgtctggacgaacaacttatcggcgtcattggccctgacggaggccattgaagctgggaccgtgtgggtcaacacgcacaatatggttgatcctaatctgccgtttggcggcttcaaagattccgggattggacgcgaacatggtgcctcggcgattgagaactatacgacgacaaaatcggtgtgcatcgcgtaccagggttga

SEQ ID NO: 58 - DNA, 1479 bp, Paraburkholderia sp. 5N
  source 1..1479: mol_type = genomic DNA
atgacagaacagaaaaccaccgcgaaactgccgactgctatgtttatcaacggcgagaaaaccctgagtgcagcgggcaagacgtttcccatctacaatcctgcgacaggtcaggaattgtcacagatcccagacgcgtcggaaaccgatattgaccatgcggtaaagaccagtaaagccgcgtttgagagtgacacttggcgccgcatgccgccggccacccgtgagcgtctgctgctgaaactcgcggacttggttgagcagcatacggacgaactggcaaccttagaaactctgaaccagggtaagctcattgtgttttccaaaatgctggaggtcactggctcagtccagtggttgcggtatatggccggttgggcaaccaaaatcgaggggacgacctttgatctgtccgtaccgtttcctccaggcacacgctacaacgcgagcaccaaacgcgttcctgccggcgttgtggcggccattgtgccatggaactttccgttattggttgctgtgtggaaaattgccccggcgttagcgtgtggctgtaccgtcgtgcttaaaccggcggaagagactccgcttaccgcaattcgtctggctgaactggctcatgaagctgggtttccgcccggggtattcaacgttgtcacaggacgtggtgaaaccgcaggggctgcactggtcaaacacccgctgattaacaaggtgacgttcacgggtagcaccgaagttggtcgcatcattggccgccaatgcgcggatgaccttaaacgcgcatctctggaactcggtggtaaatcgccggtaattgtcctggatgattgcgatccgaagaaagccattgaaggcgctgccggagcaatcttcttcaatcacggtcaagtgtgtactgccggttcgcgcctgtatgtggcccgcagcatctacgacgaagtggtgcagggtattgcagccgttgcagatgggattgccctgggcagtggttttgatgcggccacgcaaatgggccccatggtgtcagcacgtcatcgtgacaaagtgatgggcatgattgcacagggtcgccaagaaggcggagaaatcctttctcgggatgctgccgttgatgctgtggggttcttcgtgcgcccaacggtgatcgccaatcgtgcgtgcaaaccgttgagcgtagttcgcgaagaagtctttggccctgttctggtagcgatgccctatgatgacattgatgaagtgttagcgcaagcaaatgcttcggagtatggcctgggtgcgtctgtctggacgaatcagttagataaggccctccgtctggtggatggtattgaagcgggcacagtctgggttaacacgcacaatatggtcgatccagccatgccgttcggcggattcaaagcgagcggcattggacgtgaacatggcaaagcgatcgttgattcctacaccgagagcaaaagcgtatgcatcgcgtattga

SEQ ID NO: 59 - DNA, 36 bp, synthetic construct
  source 1..36: mol_type = other DNA
caccatcacggatccatgccgcatcagctgttgatt

SEQ ID NO: 60 - DNA, 37 bp, synthetic construct
  source 1..37: mol_type = other DNA
cagctaattaagcttttagtgtttgaccatgatgtgg

SEQ ID NO: 61 - DNA, 38 bp, synthetic construct
  source 1..38: mol_type = other DNA
caccatcacggatccatgcagtatcaactgctgattaa

SEQ ID NO: 62 - DNA, 38 bp, synthetic construct
  source 1..38: mol_type = other DNA
cagctaattaagcttttaatgtttcaccataatgtggc

SEQ ID NO: 63 - DNA, 37 bp, synthetic construct
  source 1..37: mol_type = other DNA
caccatcacggatccatgcacgacaaactgctgattg

SEQ ID NO: 64 - DNA, 36 bp, synthetic construct
  source 1..36: mol_type = other DNA
cagctaattaagctttcagtggcggatcatgatgtg

SEQ ID NO: 65 - DNA, 37 bp, synthetic construct
  source 1..37: mol_type = other DNA
caccatcacggatcccagagtcaattactgattaacg

SEQ ID NO: 66 - DNA, 38 bp, synthetic construct
  source 1..38: mol_type = other DNA
cagctaattaagcttctagtgttttatcattacatgcc

SEQ ID NO: 67 - DNA, 37 bp, synthetic construct
  source 1..37: mol_type = other DNA
caccatcacggatcccaaacgcagatgctgatcaatg

SEQ ID NO: 68 - DNA, 37 bp, synthetic construct
  source 1..37: mol_type = other DNA
cagctaattaagctttcaatgcttgatcatcacatgc

SEQ ID NO: 69 - DNA, 34 bp, synthetic construct
  source 1..34: mol_type = other DNA
caccatcacggatcccaacaggagcgtcgcgaag

SEQ ID NO: 70 - DNA, 36 bp, synthetic construct
  source 1..36: mol_type = other DNA
cagctaattaagctttcaaaacgggtaaatgctggg

SEQ ID NO: 71 - DNA, 36 bp, synthetic construct
  source 1..36: mol_type = other DNA
caccatcacggatccaacaccccgatcaagtcaaac

SEQ ID NO: 72 - DNA, 36 bp, synthetic construct
  source 1..36: mol_type = other DNA
cagctaattaagcttttaaaacgggtaaatgaccgg

SEQ ID NO: 73 - DNA, 34 bp, synthetic construct
  source 1..34: mol_type = other DNA
caccatcacggatcccggcggttgctggacgaac

SEQ ID NO: 74 - DNA, 34 bp, synthetic construct
  source 1..34: mol_type = other DNA
cagctaattaagctttcagaacgggtaagcgggc

SEQ ID NO: 75 - DNA, 35 bp, synthetic construct
  source 1..35: mol_type = other DNA
caccatcacggatccgcccttctcgacgaatccat

SEQ ID NO: 76 - DNA, 34 bp, synthetic construct
  source 1..34: mol_type = other DNA
cagctaattaagctttcagaaggggtaagcgggc

SEQ ID NO: 77 - DNA, 36 bp, synthetic construct
  source 1..36: mol_type = other DNA
caccatcacggatccatgaacagctcacttccgaac

SEQ ID NO: 78 - DNA, 35 bp, synthetic construct
  source 1..35: mol_type = other DNA
cagctaattaagctttcagcactgaatgtgatggc

SEQ ID NO: 79 - DNA, 37 bp, synthetic construct
  source 1..37: mol_type = other DNA
caccatcacggatccatgtatcgcgaaatttctatgc

SEQ ID NO: 80 - DNA, 34 bp, synthetic construct
  source 1..34: mol_type = other DNA
cagctaattaagctttcaaccctggtacgcgatg

SEQ ID NO: 81 - DNA, 36 bp, synthetic construct
  source 1..36: mol_type = other DNA
caccatcacggatccatgacagaacagaaaaccacc

SEQ ID NO: 82 - DNA, 35 bp, synthetic construct
  source 1..35: mol_type = other DNA
cagctaattaagctttcaatacgcgatgcatacgc

SEQ ID NO: 83 - DNA, 36 bp, synthetic construct
  source 1..36: mol_type = other DNA
caccatcacggatccatcataggggttcctaaagag

SEQ ID NO: 84 - DNA, 35 bp, synthetic construct
  source 1..35: mol_type = other DNA
cagctaattaagcttttaagcacccgccacagatg

SEQ ID NO: 85 - DNA, 39 bp, synthetic construct
  source 1..39: mol_type = other DNA
caccatcacggatccacgaatactctggatgttttaaaa

SEQ ID NO: 86 - DNA, 38 bp, synthetic construct
  source 1..38: mol_type = other DNA
cagctaattaagcttttacagccaagttgatacttttg

SEQ ID NO: 87 - DNA, 23 bp, synthetic construct
  source 1..23: mol_type = other DNA
catggtatatctccttcttaaag

SEQ ID NO: 88 - DNA, 18 bp, synthetic construct
  source 1..18: mol_type = other DNA
ctcgagcaccaccaccac

SEQ ID NO: 89 - DNA, 40 bp, synthetic construct
  source 1..40: mol_type = other DNA
taagaaggagatataccatgaacaggttaccttcgagcgc

SEQ ID NO: 90 - DNA, 41 bp, synthetic construct
  source 1..41: mol_type = other DNA
catggtatatctccttcttattacgcttcttcgacacttac

SEQ ID NO: 91 - DNA, 39 bp, synthetic construct
  source 1..39: mol_type = other DNA
taagaaggagatataccatgcgtgagaccaaggagcaac

SEQ ID NO: 92 - DNA, 40 bp, synthetic construct
  source 1..40: mol_type = other DNA
tggtggtggtggtgctcgagttaaaacgggtagttcgccg

SEQ ID NO: 93 - DNA, 39 bp, synthetic construct; identical to SEQ ID NO: 91
  source 1..39: mol_type = other DNA

SEQ ID NO: 94 - DNA, 40 bp, synthetic construct
  source 1..40: mol_type = other DNA
catggtatatctccttcttattaaaacgggtagttcgccg

SEQ ID NO: 95 - DNA, 40 bp, synthetic construct; identical to SEQ ID NO: 89
  source 1..40: mol_type = other DNA

SEQ ID NO: 96 - DNA, 41 bp, synthetic construct
  source 1..41: mol_type = other DNA
tggtggtggtggtgctcgagttacgcttcttcgacacttac

SEQ ID NO: 97 - DNA, 21 bp, synthetic construct
  source 1..21: mol_type = other DNA
catagctgtttcctgtgtgaa

SEQ ID NO: 98 - DNA, 20 bp, synthetic construct
  source 1..20: mol_type = other DNA
gaattcactggccgtcgttt

SEQ ID NO: 99 - DNA, 40 bp, synthetic construct
  source 1..40: mol_type = other DNA
tcacacaggaaacagctatgaacaggttaccttcgagcgc

SEQ ID NO: 100 - DNA, 40 bp, synthetic construct
  source 1..40: mol_type = other DNA
aaacgacggccagtgaattcttaaaacgggtagttcgccg

SEQ ID NO: 101 - DNA, 39 bp, synthetic construct
  source 1..39: mol_type = other DNA
tcacacaggaaacagctatgcgtgagaccaaggagcaac

SEQ ID NO: 102 - DNA, 41 bp, synthetic construct
  source 1..41: mol_type = other DNA
aaacgacggccagtgaattcttacgcttcttcgacacttac

SEQ ID NO: 103 - protein, 454 aa, Pseudomonas chlororaphis subsp. aureofaciens NBRC 3521
MTSNNPQTREWQTLSSEHHLAPFSDFKQLKEKGPRIITNAEGVYLWDSEGNKILDGMAGLWCVAIGYGREELADAASKQMRELPYYNLFFQTAHPPALELAKAISDVAPQGMNHVFFTGSGSEGNDTMLRMVRHYWAIKGQPKKKTIISRVNGYHGSTVAGASLGGMTYMHEQGDLPIPGIVHIPQPYWFGEGGDMTPDEFGIWAANQLEEKILELGVDNVGAFIAEPIQGAGGVIVPPESYWPRIKEILAKYDILFVADEVICGFGRTGEWFGSDFYDLKPDMMTIAKGLTSGYIPMGGLIVRDEVVAVLNEGGDFNHGFTYSGHPVAAAVALENIRIMRDEKIIERVKAETAPYLQKRLRELNDHPLVGEVRGVGLLGAIELVQDKATRARYVGKGVGMICRQFCFDNGLIMRAVGDTMIIAPPLVITKEEIDELVSKARKCLDLTLSALQG

SEQ ID NO: 104 - protein, 456 aa, Pseudomonas aeruginosa PAO1
MNSQITNAKTREWQALSRDHHLPPFTDYKQLNEKGARIITKAEGVYIWDSEGNKILDAMAGLWCVNVGYGREELVQAATRQMRELPFYNLFFQTAHPPVVELAKAIADVAPEGMNHVFFTGSGSEANDTVLRMVRHYWATKGQPQKKVVIGRWNGYHGSTVAGVSLGGMKALHEQGDFPIPGIVHIAQPYWYGEGGDMSPDEFGVWAAEQLEKKILEVGEENVAAFIAEPIQGAGGVIVPPDTYWPKIREILAKYDILFIADEVICGFGRTGEWFGSQYYGNAPDLMPIAKGLTSGYIPMGGVVVRDEIVEVLNQGGEFYHGFTYSGHPVAAAVALENIRILREEKIIEKVKAETAPYLQKRWQELADHPLVGEARGVGMVAALELVKNKKTRERFTDKGVGMLCREHCFRNGLIMRAVGDTMIISPPLVIDPSQIDELITLARKCLDQTAAAVLA

SEQ ID NO: 105 - protein, 462 aa, Halomonas elongata DSM 2581
GMQTQDYQALDRAHHLHPFTDFKALGEEGSRVVTHAEGVYIHDSEGNRILDGMAGLWCVNLGYGRRELVEAATAQLEQLPYYNTFFKTTHPPAVRLAEKLCDLAPAHINRVFFTGSGSEANDTVLRMVRRYWALKGQPDKQWIIGRENAYHGSTLAGMSLGGMAPMHAQGGPCVPGIAHIRQPYWFGEGRDMSPEAFGQTCAEALEEKILELGEEKVAAFIAEPVQGAGGAIMPPESYWPAVKKVLAKYDILLVADEVICGFGRLGEWFGSQHYGLEPDLMPIAKGLSSGYLPIGGVLVGDRVAETLIEEGGEFFHGFTYSGHPTCAAVALKNLELLEAEGVVDRVRDDLGPYLAERWASLVDHPIVGEARSLGLMGALELVADKTTGQRFDKSLGAGNLCRDLCFANGLVMRSVGDTMIISPPLVIRREEIDELVELARRALDETARQLTQVPHTQEEPTA

SEQ ID NO: 106 - protein, 469 aa, Halomonas elongata DSM 2581
MTTHKDLIDRDRKVTFHASTHLRDFAHGDAPGRVITGGKGIKIVDKDGREFIDGFAGLYCVNIGYGRSEVAEAIYQQALEMSYYHTYVGHSNEPQIALSEKILELAGPGMSKVYYGMSGSDANETQLKIVRYYNNVLGRPQKKKVISRMRGYHGSGIASGSLTGLKAFHDHFDLPIETIRHTEAPYYYHRAAEQEGMTEREFSKHCAAKLEEMILAEGPDTVAAFIGEPVLGTGGIVPPPEGYWDEIQAVLTKYDVLLIADEVVCGFGRTGSDFGSHHYGIKPDLITIAKGLTSAYQPLSGVIVGDRVWEVLEQGTGEYGPIGHGWTYSGHALGCAAGLANLAIIEREGLTANAAETGAYLQERMKAAFADHPVVGQVRGVGMMAALEFSVDPAARRHFDPSLKVGPRMSAAALEEDLIARAMPQGDILGFAPPLTTTREEVDEIVARTERAVNKVTDALTREGAIQAA

SEQ ID NO: 107 - protein, 395 aa, Methanosarcina acetivorans C2A
METRTLEDWRALLEAEKTLDSGVYNKHDLLIVRGQGARVWDAEGNEYIDCVGGYGVANLGHGNPEVVEAVKRQAETLMAMPQTLPTPMRGEFYRTLTAILPPELNRVFPVNSGTEANEAALKFARAHTGRKKFVAAMRGFSGRTMGSLSVTWEPKYREPFLPLVEPVEFIPYNDVEALKRAVDEETAAVILEPVQGEGGVRPATPEFLRAAREITQEKGALLILDEIQTGMGRTGKRFAFEHFGIVPDILTLAKALGGGVPLGVAVMREEVARSMPKGGHGTTFGGNPLAMAAGVAAIRYLERTRLWERAAELGPWFMEKLRAIPSPKIREVRGMGLMVGLELKEKAAPYIARLEKEHRVLALQAGPTVIRFLPPLVIEKEDLERVVEAVRAVLA

SEQ ID NO: 108 - DNA, 1365 bp, Pseudomonas chlororaphis subsp. aureofaciens NBRC 3521
  source 1..1365: mol_type = genomic DNA
atgaccagcaacaacccgcaaacccgtgagtggcaaaccctcagcagcgagcaccacctggcacccttcagcgacttcaagcagttgaaggagaaggggccgcggatcatcactaatgccgagggcgtttacctctgggacagcgagggcaacaagatcctcgacggtatggccgggctgtggtgcgtggccatcggttacggccgcgaagaactggccgacgccgccagcaagcagatgcgcgagctgccgtactacaacctgttcttccagaccgcccacccgccggcgctggaactggccaaggccatctccgatgttgctccgcagggcatgaaccatgtgttcttcaccggttccggctccgaaggcaacgacaccatgctgcgcatggttcgccactactgggcgatcaagggccagccgaagaagaaaaccatcatcagccgggtcaacggctatcacggttccaccgtggccggcgcgagcctgggcggcatgacctatatgcacgaacagggcgacttgccgatcccaggcatcgtgcatatcccgcagccttactggttcggtgaaggcggcgacatgaccccggacgagttcgggatctgggcggccaaccagctggaagagaagattctcgaactcggcgtcgacaacgtcggtgccttcattgccgagccgatccagggcgcgggcggcgtgatcgtgccgccggaaagctactggccgcggatcaaggagatccttgccaagtacgacatcctgttcgtcgccgacgaggtgatctgtgggttcgggcgtaccggtgagtggttcggtagcgatttctacgacctcaagccggacatgatgactatcgccaagggcctgacttccggctacatccccatgggtggcctgatcgtgcgcgacgaagtggtggcggtgctcaacgagggcggcgatttcaaccacggtttcacctattccgggcacccggtggccgccgccgtggccctggaaaacatccgcatcatgcgcgacgagaaaattatcgagcgcgtcaaggcagaaacggcaccttatttgcagaaacgtctgcgggaactgaacgatcacccgctggtgggtgaggttcgcggagtcggcctgttgggcgccatcgaactggttcaggacaaggccacccgtgcgcggtatgtcggaaaaggcgtcggcatgatctgccggcagttctgcttcgacaacggcctgatcatgcgcgccgtgggcgacaccatgatcattgctccgcccctggtgatcaccaaggaggagatcgatgagctggtgagcaaggcccgcaagtgcctggacctgaccttgagtgcgttgcagggctaa

SEQ ID NO: 109 - DNA, 1371 bp, Pseudomonas aeruginosa PAO1
  source 1..1371: mol_type = genomic DNA
atgaacagccaaatcaccaacgccaagacccgtgagtggcaggcgttgagccgcgaccaccatctgccgccgttcaccgactacaagcagttgaacgagaagggcgcgcggatcatcaccaaggccgaaggcgtctatatctgggacagcgagggcaacaagatcctcgatgcgatggccggcctctggtgcgtcaacgtcggctacggccgcgaggagctggtccaggccgccacccggcagatgcgcgagttgccgttctacaacctgttcttccagaccgcccacccgccggtggtcgagctggccaaggcgatcgccgacgtcgctccggaaggcatgaaccacgtgttcttcaccggctccggctccgaggccaacgacaccgtgctgcgtatggtccgccactattgggcgaccaagggccagccgcagaagaaagtggtgatcggccgctggaacggctaccacggctccaccgtcgccggcgtcagcctgggcggcatgaaggcgttgcatgagcagggtgatttccccatcccgggcatcgtccacatcgcccagccctactggtacggcgagggcggcgacatgtcgccggacgagttcggcgtctgggccgccgagcagttggagaagaagattctcgaagtgggcgaggaaaacgtcgccgccttcatcgccgagccgatccagggcgccggcggcgtgatcgtcccgccggacacctactggccgaagatccgcgagatcctcgccaagtacgacatcctgttcatcgccgacgaagtgatctgcggcttcggccgtaccggcgagtggttcggcagccagtactacggcaacgccccggacctgatgccgatcgccaagggcctcacctccggctacatccccatgggcggggtggtggtgcgcgacgagatcgtcgaagtgctcaaccagggcggcgagttctaccacggcttcacctattccggtcacccggtggcggccgccgtggccctggagaacatccgcatcctgcgcgaagagaagatcatcgagaaggtgaaggcggaaacggcaccgtatttgcagaaacgctggcaggagctggccgaccacccgttggtgggcgaagcgcgcggggtcggcatggtcgccgccctggagctggtcaagaacaagaagacccgcgagcgtttcaccgacaagggcgtcgggatgctgtgccgggaacattgtttccgcaacggtttgatcatgcgcgcggtgggcgacactatgattatctcgccgccgctggtgatcgatccgtcgcagatcgatgagttgatcaccctggcgcgcaagtgcctcgatcagaccgccgccgccgtcctggcttga

SEQ ID NO: 110 - DNA, 1386 bp, Halomonas elongata DSM 2581
  source 1..1386: mol_type = genomic DNA
atgcaaacccaagactatcaggccctggaccgcgcccatcacctgcatcccttcaccgatttcaaggcgttgggtgaagagggcagtcgcgtcgtgacccacgccgaaggcgtctacatccacgacagcgagggcaaccgcattctcgacggcatggccgggctttggtgcgtgaatctcggctatggtcgccgcgaactggtcgaggcggcaacggcgcagctcgagcaactgccgtactacaacaccttcttcaagaccacgcatccgcccgcggtgcgcctggccgagaagctgtgcgatctagcgccggcgcacatcaatcgtgtgttcttcaccggctccggttccgaggccaacgacaccgtgctgcgcatggtacggcgttactgggccttgaagggccaacccgacaagcaatggatcatcggtcgcgagaacgcctatcacggctccaccctggccggcatgagcctgggcggcatggcgccgatgcatgcccagggcggcccctgcgtgcccggcatcgcccacatccgccagccctactggttcggcgaggggcgggacatgtcgccggaggccttcggccagacgtgcgctgaggcgctggaggagaaaatcctcgagctcggcgaggagaaggtggccgctttcatcgccgaaccggtgcagggcgccgggggggccatcatgccgccggagagctactggccggccgtcaagaaagtgctggcgaaatacgacatcctgctggtcgccgacgaggtgatctgcggcttcgggcgactcggcgagtggttcggcagccagcactacggtctcgagcccgacctgatgccgatcgccaagggcctgtcctccggctatctaccgatcggcggcgtgctggtcggggatcgtgtcgccgagacgctgatcgaagaaggcggcgagttcttccacggtttcacctactcggggcatccgacctgtgccgccgtggcgctcaaaaacctcgagctactcgaggccgagggcgtggtggatcgggtgcgcgacgatcttggtccctatctggccgagcgctgggccagcctggtcgaccatcctatcgtcggcgaggcacgatccctgggcctgatgggtgccctggaactggtcgccgacaagaccaccgggcagcgtttcgacaagtcgctgggcgccggcaacctgtgccgtgacctgtgcttcgccaatggcctggtgatgcgctccgtgggcgataccatgatcatttcgccaccgctggtgattcgtcgcgaggaaatcgacgaactggtggaactggcccgacgggccctggacgagacggctcgccaactgacgcaagtgccgcacacgcaagaggagccaaccgcatga

SEQ ID NO: 111 - DNA, 1410 bp, Halomonas elongata DSM 2581
  source 1..1410: mol_type = genomic DNA
atgaccactcacaaggatctgatcgatcgcgaccgcaaggtgaccttccacgcctccacccacctgcgcgacttcgcccatggcgacgcgccgggccgggtgatcaccggcggcaagggcatcaagatcgtcgacaaggacggccgcgagttcatcgacggcttcgccggcctgtattgcgtcaacatcggctacggccgcagcgaggtcgccgaggcgatttatcagcaggccctggagatgtcctactaccatacctatgtgggccactccaacgagccgcagatcgcgctttccgagaagatcctcgagctggccggccccggcatgtccaaggtctactacggcatgtccggcagcgacgccaatgagacccagctcaagatcgtgcgttactacaacaacgtgctcggccgcccgcagaagaagaaagtcatctcgcgcatgcgcggctatcacggctccggcatcgcctccggctcgctgaccgggctgaaggcgttccacgatcatttcgacctgccgatcgagacgatccgccacaccgaggcgccgtactactatcatcgtgccgccgagcaggaaggcatgaccgagcgcgagttctccaagcattgtgccgccaagctggaggagatgatcctggccgaaggaccggacaccgtggctgccttcatcggcgagccggtgctcggcaccggcggcatcgtgccgccgcccgaaggctactgggacgagatccaggcggtgctgaccaagtacgacgtgctgctgatcgccgacgaagtggtgtgcggcttcggtcgcacgggcagcgacttcggcagccatcactacggcatcaagccggacctgatcaccatcgccaagggcctgaccagcgcctatcagccgctctccggggtgatcgttggcgaccgcgtctgggaagtgctcgagcagggcaccggcgaatacggcccgatcggccacggctggacctattccggccacgccctgggctgtgccgccgggctggccaacctggcgatcatcgaacgcgaaggcctcaccgccaacgccgccgagaccggcgcctacctgcaggagcgcatgaaggctgccttcgccgaccatccggtcgtcggccaggtgcgtggcgtgggcatgatggcggcgctggagttttccgtcgacccggcggcgcgtcgtcacttcgatccgtccctcaaggtcgggccgcgcatgtccgccgccgccctcgaggaagacctgatcgcacgcgccatgccgcagggcgatatcctcggcttcgcgccgccgctgaccaccactcgcgaggaagtcgacgagatcgtcgcgcgcaccgagcgggcggtgaacaaggtgaccgatgcgctgacgcgggaaggtgccatccaggccgcctga

SEQ ID NO: 112 - DNA, 1188 bp, Methanosarcina acetivorans C2
  source 1..1188: mol_type = genomic DNA
gtggaaacgagaaccctggaagactggcgggcccttttggaggcggagaagaccctggacagcggcgtctacaacaagcacgacctcctcatcgtccggggccagggcgcgagggtctgggacgcggaaggcaacgagtacattgactgcgtgggcgggtacggggtggccaacctgggccacggcaaccccgaggtggtggaggcggtgaagcggcaggcggagacccttatggccatgccccagaccctccccacccccatgcggggggagttctaccgcaccctcaccgccatcctccccccggagctcaaccgggtcttccccgtgaactcgggcaccgaggccaacgaggccgccctaaagttcgcccgggcccacacgggcaggaagaagttcgtggccgccatgcggggcttctccgggcgaaccatgggaagcctctccgtcacctgggagcccaagtaccgggagcctttcttgcccttggtggagcccgtggagttcatcccctacaacgacgtggaggccctcaagcgggccgtggacgaggagacggccgcggtgatcctggagcccgtgcaaggggaggggggcgtgcgcccggcgacccccgagttcctaagggccgcccgggagatcacccaggagaagggggccctcctcatcctggacgagatccagaccggaatgggccgcacggggaagcgcttcgcctttgagcacttcggcatcgtccccgacatcctcaccctggccaaggccctcgggggcggggtgcccctgggggccgcggtgatgcgggaggaggtggcgcggagcatgcccaagggggggcacggcaccaccttcggggggaatcccctggccatggccgcaggggtggcggccatccgctacctggagcggacgcggctttgggaaagggccgcggagcttgggccctggttcatggagaagcttagggccatcccctcccccaagatccgggaggtgcggggcatgggcctcatggtgggcctggagctcaaggaaaaggccgccccctacatcgccaggctggagaaggagcaccgcgtcctcgccctccaggctgggcccacggtgatccgcttcctgccgcctttggtcattgaaaaggaagacctggagcgggtggtggaggcggtgcgggcggtgctagcatag

SEQ ID NO: 113 - DNA, 35 bp, synthetic construct
  source 1..35: mol_type = other DNA
caccatcacggatccaccagcaacaacccgcaaac

SEQ ID NO: 114 - DNA, 34 bp, synthetic construct
  source 1..34: mol_type = other DNA
cagctaattaagcttttagccctgcaacgcactc

SEQ ID NO: 115 - DNA, 35 bp, synthetic construct
  source 1..35: mol_type = other DNA
caccatcacggatccaacagccaaatcaccaacgc

SEQ ID NO: 116 - DNA, 33 bp, synthetic construct
  source 1..33: mol_type = other DNA
cagctaattaagctttcaagccaggacggcggc

SEQ ID NO: 117 - DNA, 35 bp, synthetic construct
  source 1..35: mol_type = other DNA
caccatcacggatcccaaacccaagactatcaggc

SEQ ID NO: 118 - DNA, 35 bp, synthetic construct
  source 1..35: mol_type = other DNA
cagctaattaagctttcatgcggttggctcctctt

SEQ ID NO: 119 - DNA, 36 bp, synthetic construct
  source 1..36: mol_type = other DNA
caccatcacggatccaccactcacaaggatctgatc

SEQ ID NO: 120 - DNA, 33 bp, synthetic construct
  source 1..33: mol_type = other DNA
cagctaattaagctttcaggcggcctggatggc

SEQ ID NO: 121 - DNA, 39 bp, synthetic construct
  source 1..39: mol_type = other DNA
caccatcacggatccatcacaaattcaaggaaaggaatt

SEQ ID NO: 122 - DNA, 36 bp, synthetic construct
  source 1..36: mol_type = other DNA
cagctaattaagctttcaggcctgctcaagaacatc

SEQ ID NO: 123 - protein, 378 aa, Bacillus subtilis 168
MIIGVPKEIKNNENRVALTPGGVSQLISNGHRVLVETGAGLGSGFENEAYESAGAEIIADPKQVWDAEMVMKVKEPLPEEYVYFRKGLVLFTYLHLAAEPELAQALKDKGVTAIAYETVSEGRTLPLLTPMSEVAGRMAAQIGAQFLEKPKGGKGILLAGVPGVSRGKVTIIGGGVVGTNAAKMAVGLGADVTIIDLNADRLRQLDDIFGHQIKTLISNPVNIADAVAEADLLICAVLIPGAKAPTLVTEEMVKQMKPGSVIVDVAIDQGGIVETVDHITTHDQPTYEKHGVVHYAVANMPGAVPRTSTIALTNVTVPYALQIANKGAVKALADNTALRAGLNTANGHVTYEAVARDLGYEYVPAEKALQDESSVAGA

SEQ ID NO: 124 - DNA, 1137 bp, Bacillus subtilis 168
  source 1..1137: mol_type = genomic DNA
atgatcataggggttcctaaagagataaaaaacaatgaaaaccgtgtcgcattaacacccgggggcgtttctcagctcatttcaaacggccaccgggtgctggttgaaacaggcgcgggccttggaagcggatttgaaaatgaagcctatgagtcagcaggagcggaaatcattgctgatccgaagcaggtctgggacgccgaaatggtcatgaaagtaaaagaaccgctgccggaagaatatgtttattttcgcaaaggacttgtgctgtttacgtaccttcatttagcagctgagcctgagcttgcacaggccttgaaggataaaggagtaactgccatcgcatatgaaacggtcagtgaaggccggacattgcctcttctgacgccaatgtcagaggttgcgggcagaatggcagcgcaaatcggcgctcaattcttagaaaagcctaaaggcggaaaaggcattctgcttgccggggtgcctggcgtttcccgcggaaaagtaacaattatcggaggaggcgttgtcgggacaaacgcggcgaaaatggctgtcggcctcggtgcagatgtgacgatcattgacttaaacgcagaccgcttgcgccagcttgatgacatcttcggccatcagattaaaacgttaatttctaatccggtcaatattgctgatgctgtggcggaagcggatctcctcatttgcgcggtattaattccgggtgctaaagctccgactcttgtcactgaggaaatggtaaaacaaatgaaacccggttcagttattgttgatgtagcgatcgaccaaggcggcatcgtcgaaactgtcgaccatatcacaacacatgatcagccaacatatgaaaaacacggggttgtgcattatgctgtagcgaacatgccaggcgcagtccctcgtacatcaacaatcgccctgactaacgttactgttccatacgcgctgcaaatcgcgaacaaaggggcagtaaaagcgctcgcagacaatacggcactgagagcgggtttaaacaccgcaaacggacacgtgacctatgaagctgtagcaagagatctaggctatgagtatgttcctgccgagaaagctttacaggatgaatcatctgtggcgggtgcttaa

SEQ ID NO: 125 - protein, 202 aa, Bacillus subtilis 168
MTNTLDVLKARASVKEYDTNAPISKEELTELLDLATKAPSAWNLQHWHFTVFHSDESKAELLPVAYNQKQIVESSAVVAILGDLKANENGEEVYAELASQGYITDEIKQTLLGQINGAYQSEQFARDSAFLNASLAAMQLMIAAKAKGYDTCAIGGFNKEQFQKQFDISERYVPVMLISIGKAVKPAHQSNRLPLSKVSTWL

SEQ ID NO: 126 - DNA, 609 bp, Bacillus subtilis 168
  source 1..609: mol_type = genomic DNA
atgacgaatactctggatgttttaaaagcacgtgcatctgtaaaggaatatgatacaaatgccccgatctctaaggaggagctgactgagctattagaccttgccactaaagcgccttctgcttggaaccttcagcattggcattttacagtattccacagcgatgaatcaaaagcggagcttcttcctgtagcgtataatcaaaaacaaatcgttgagtcttctgctgttgttgccattttaggcgatttaaaggcaaatgaaaacggtgaagaagtttatgctgaattagcaagccaaggctatattacggatgaaatcaaacaaacattgctcggccaaatcaacggtgcttaccaaagcgagcaattcgcacgtgattccgctttcttaaatgcttctttagctgctatgcagcttatgattgccgcaaaagcaaaaggttatgacacttgcgcaatcggcggatttaacaaagagcagttccaaaagcaatttgatatcagtgagcgctatgttccggttatgcttatttcaatcggcaaagcagtgaagcctgcgcatcaaagcaaccgtctgccgctttcaaaagtatcaacttggctgtaa

SEQ ID NO: 127 - protein, 487 aa, Hydrogenophaga aromaticivorans
MNTPVKTERWSGKIFTGSWVAARGGVAPVLEAATGAALGEVGVASPEDVDAAARSAQAAQKAWAATPFDQRAAIVREAARLLKERAAEFTQWNVRECGSIVPKGEWEVGITHEQMQQAAALAGLPNGMMFPSSVPGRTNLWQRVPLGVVGVIAPWNFPLFLAMRSVAPALALGNAVLLKPDLQSAVTGGALIARLFEDVGLPPGVLQVLPGGPATGDAVVRHPCVNMVSFTGSTAVGRQIGEFCGRALKKVALELGGNNAMIVLDDADLDGASSCAAWGGFLHQGQICMAAGRHLVHRSVADAYAAKLVERAKKLYVGDPHAGPAHLGPLINDRQTERVHRIVTESIAAGATLLAGGTHEGRFYQPTVLSNVAVDMPAFAEEIFGPVAPITVFDTDEEAVALANSSEYGLAAAIHSKSTARALRMASQLKSGMVHINDQPVNCEPQVPFGGMGASGSGGRFGGPASIDEFTQAQWVSVSEKAAQYPF

SEQ ID NO: 128 - protein, 487 aa, Pseudomonas aeruginosa
MRETKEQPIWYGKVFSSNWVEARGGVANVVDPSNGDILGITGVANGEDVDAAVNAAKRAQKEWAAIPFSERAAIVRKAAEKLKEREHEFADWNVRECGAIRPKGLWEAGIAYEQMHQAAGLAYLSNGTLFPSAVPGRMNLCQRVPVGVVGVIAPWNFPLFLAMRSVAPALALGNAVILKPDLQTAVTGGALIAEIFSDAGMPDGVLHVLPGGADVGESMVANSGINMISFTGSTQVGRLIGEKCGRMLKKVALELGGNNVHIVLPDADLDGAVSCAAWGTFLHQGQVCMAAGRHLVHRDVAQQYAEKLALRAKNLVVGDPNSDRVHLGPLINDKQVVRVHALVESAQSAGAKVLAGGTYQDRYYQATVIMDVKPEMEVFKSEIFGPVAPITVFDSIEEAIELANCSEYGLAASIHTRALATGLDIAKRLNTGMVHINDQPINCEPHVPFGGMGSSGSGGRFGGLASIDEFTQSQWISMVEKSASYPF

SEQ ID NO: 129 - protein, 487 aa, Pseudomonas sp. MAP12
MHETKEQPIWGGKIFSSTWVEARGGVANVVDPSNGDILGITGVANREDVDVAVSAAKIAQKEWAAMPFSERAAIVRKAADKLKEREHEFADWNVRECGAIRPKGLWEAGITYEQMHQAVGLASLPNGALFPSAVSGRMNLCQRVPIGVVGVIAPWNFPLFLAMRSVAPALVLGNAVVLKADLQTAVIGGALIAEIFSDAGIPEGVLHVLPGGADVGESMVENPGINMISFTGSTQVGRSIGEKCGRMLKKVSLELGGNNVNIVLPDADLDGAVGCAAWGTFFHQGQVCMAAGRHLVHRDIAQEYAAKLAKRAQSLVVGDPNTDQVHLGPLINDKQVDRVHALVESAERAGAKVLAGGAYEGRYYQATVVMDVKPDMEIFQSEIFGPVAPITIFDSIDEAIELANSSEYGLAASIHTKSLTTGMKIANRLKTGMVHINDQPINCEPHVPFGGMGASGSGGRFGGTASIEEFTQSQWISVVDKTAVYPF

SEQ ID NO: 130 - protein, 489 aa, Alteromonas
MQQERKKEVPIWSGKVFSSGWVEARGGASDVTDPSNGDLLGVVGIANGEDVAAAAQSARRAQKEWAAIPFSERAEIVRKAAEKLKERENEFADWNVRECGAIRQKGLWEAGITYQQMHQAASLAFLPDGTSLPSTVAGRLNLCHRVPVGVVGVIAPWNFPLFLAMRSVAPALVLGNAVILKPDPQTAVTGGALIAEIFSEAGIPDGVIHVLPGGAEAGESMVTNPGIDMISFTGSTEVGRLIGEKCGRMLKKVALELGGNNVHIILPDADLDGAASCAAWGTFLHQGQVCMAAGRHLVHRDIAQEYAEKLALRARNLVVGDPKTDQVHLGPLVNDKQVAHVHALVESAQKAGAKILAGGTYQDRYYQATVLMDVTPKMDIFELETFGPVAPITIVDSVEEAIGLANSSEYGLAASIHTKDLAAGLEIARNLKTGMVHINDQPINCEPHVPFGGMGASGSSGRFGGLASIDAFTQSQWISMVGKPATYPF

SEQ ID NO: 131 - protein, 487 aa, Tepidiphilus succinatimandens
MNWNGKLPIWHGKVFSNGWVVPRGGVADVVDPSSGDVLGVTGIANSEDIATAASAAKEAQKKWAAMPFNDRAAILRKAAEKLREREAEFADWNVRECGAVRMKGVWEAGITYEQMHQAASLAFLPNGTLFPSQVPGRMNFVHRVPVGVVGVIAPWNFPLFLAMRSVAPALVLGNAVILKPDVQTAVTGGALIAEIFAEAGIPEGVLHVLPGGADAGDAMVTNPEIDMISFTGSTAVGRQIGEKCGRMLKKVTLELGGNNVHIVLPDADLTGAASCAAWGTFLHQGQVCMAAGRHLVHRDVAQQYAQELAARAKNLVVGDPKTDQVHLGPLINDKQVARVHALVESAQKQGAKVLVGGTHQGRFYQPTVLMDVRPDMDVFKSEIFGPVAPITVFDTIDEAIELANSSEYGLAASIHTSAIATALQIAKRLKTGMVHINDQPINCEPHVPFGGMGASGTSGRFGGLSSIDEFTQSQWISMVEKPTNYPF

SEQ ID NO: 132 - protein, 487 aa, Halomonas cupida
MSTFFNAETYSNRIYLNDWRESRGGTSDVVEPATGKVLARTAIGNSEDIREAIVEAKAQQPAWARLPFDQRARILRRAAELLLEHRDTFIEWNIRECGSIVPKAEAELHSTHEQLNMAAAMTMQPDGITLPSSMPGRRNTCRRVPLGVVGVITPWNFPLLLAMRSVAPAIAVGNSVVLKPDHQSAVTGGLLIARLFEEAGLPAGVLQVIPGGAEAGEALVTHPLTAMISFTGSTAVGRKIGRTCGELLKKSALELGGNNAFIVLDDADIDAAASHGAWGAYLHQGQICMQSGRHFVHHSVAEAYISKLAERAERLTVADPFLGTADIGPLINAQQLEKLDMAVTASINDGARLVTGGHSHGQFYRPTVLSNVSIDMPAFQQELFGPVAPVTTFHDEEELIEKVSASSYGLAAAIHSSSIGRALDLAERIPAGMIHINDQTVNNEFQVPFGGFGDSGNSGRFGGPANLEEFTQSQWVSLMNTPRTYPF

SEQ ID NO: 133 - protein, 498 aa, Pseudomonas fluorescens
MTTANLHNQYPSIAEFIAEHRWKACFYPGAWESAEREIPVFEPATGERLASVGIASAAEVARAGLRARQAQPAWAATPFDQRAAILREAARLLQQEAESFIEWNIRECGGARFKAEWELNICVEQLQMAAAMPMQANGELFPSSMPGRTNIWRRVPMGVVAVISPWNFPLLLSLRSIAPALALGNAVLLKPSEFSSVTGGLLLARLFELAGVPQGVFQVLPGLAETGSALVSDPCVKMVAFTGSTAVGRRIAETCGGLLKRCSLELGGNNALIVCPDADLDAASSSGAWGSFLHQGQICMQAGRHIVHRSVVAAYTEKLKDRAERLACGNPFTEAVQLGPLINAQQRDRVHGLVQDAVHQGATLVTGGEYKELCYRPTVLIGVTPDMPVFKDEIFGPVAPIVVYDDIEEALALVNASPYGLAVAIHTGNATRGYEWAGRIHSGMVHVNDQTVNNEFQVPFGGMGASGYGGRYGGPANFDEFTERQWVSLTSDPIQYPF

SEQ ID NO: 134 - protein, 487 aa, Glaciimonas immobilis
MNTSTVTNIWDSKIYSGGWIAAEGGTAAIIEPATEQVLGHIGIGATQDVDRAVQIASHAQRSWARMPFDQRANIMREAARLVLERAAEFNVWNIRQCGSIPAKAEWELHATCEQILMAAALPMQPEGLLFPSSMPGRTNLSRQLPIGVIGVITPWNFPLLLAMRSVAPALALGNAVILKPDQQSAICGGALIAQAFEDAGLPVGVLHVIPGGPATGDALVKHPEVGMISFTGSTAVGRAIGQTCGYLLKKVALELGGNNAIIVLDDADMDAASSNGAWGAFLHQGQICMQTGRHLVHHSVADQYAEKLAARAEKLHVGNPHTDQVHLGPLINRKQCDRIHGIVQETLRAGAHALTGATHERLFYRPTVLTGVTPDMAAFQEELFGPVAPVTVFHDDDEAVELVNRSAYGLCAAIHSRNIPRAVALSQRLNTGMIHINDQTVNNEFHVPFGGMGSSGNGGRFGGPANVHEFTQSQWLSIMEKPVIYPF

SEQ ID NO: 135 - protein, 487 aa, Paraburkholderia unamae
MTGTGSEGQWTGKIFLGEWVKGTGATAPVMEPATDNQIGTIALASREDVDTAIERAVVAQRAWAETTFDKRAAVLHEAARLIKARAERFNYWNVRECGSIVPKAQWELDASYEQLLMAAALPMHPTGTLFPSSMPGRTNTWRRLPIGVVGVIAPWNFPLLLALRSVAPAIALGNAVVLKPDQQSAVTGGALIAELFEDAGLPRGVLQVLPGGAQTGDAVVRHPAVGMISFTGSTAVGRQIGETCGRMLKKTSLELGGNNPIIVLPDADLDKAASCAAWGAFLHQGQICMQAGRHLVHRSVAESYVAKLAARARKLAVGNPATEPVHIGPLINARQAERVERIVRDSVEMGAVIAAGGQRRGRFFEPTVLADVTPHMPAFKDEIFGPVAPVTLFDSVDEAIELVHASEYGLAAAVHSGSMSAAMSVARRLKSGMIHINDQTVNNEFQVPFGGMGASGNGGRFGGPANVEEFTQTQWISAMDAPIEYPF

SEQ ID NO: 136 - protein, 486 aa, Marinobacter salsuginis
MDMPASPVWQEQLFLGSWKSGDGDQINVVEPATGAVISKLKIATAGDVERAATIARDTQTAWAMVPFDQKAEILRKAAALLKERANEINDWNTRECGSVGPKADWELQATYEQAQMAAALPMQPNGEIFPSNMPGKRNYWKRVPIGTVGVIAPWNFPILLAMRSVFPALAMGNAVILKPDPKSSICGGALMAQILSDAGLPEGVFHVLPGGPEVGQALVEHPLVKMISFTGSTAVGRKIGETCGRTLKKAALELGGNNAQVVLEDADLDIASSCGAWGAFLHQGQICMQTGRHLVHTSVAEEYLSRLASRAENLACGNPAQEQVHQGPLINGVQAKRVEDIVNRSVEMGARIVTGGKRHGNYYEPTVITDVTSNMPVFSEEVFGPVAPVMTFDSDSEACELVNESPYGLAAAIHSGSTERALKIANRIQVGMIHINDQTVNNEFQVPFGGMGSSGNSGRFGGPANIEEFTTSQWISVMEEGIQYPF

SEQ ID NO: 137 - protein, 486 aa, Aromatoleum toluclasticum
MNDRNTTRWHQRIFVGEWTPGRGDTVPVIEPATGDQLALLSTASIEDVDAAARLAAEAQPAWAALPFDRRAAVLRKVAQLLQERAAEINHWNIRECGSIPPKAEWELNATIEQAHMAAAMPMQPIGEIFPSSMPGRRNYWQRLPIGVVGVIAPWNFPILLGLRSVLPALAMGNAVILKPDLQSAICGGLLLAEVFEDAGLPKGVFHVLPGGPVTGDALVRHPRVKMISFTGSTAVGRLIGETCGRMLKKVALELGGNNAMVILDDADLESASSCAAWGAFLHQGQICMQAGRHLVHRKVADRYAELLAVRAAKLVVGNPATGPVHLGPLINDRQAAKVAEVVERSAALGARVLAGGKRDGRFFPATVLAGVTPDMPAYTEEIFGPVAPITVFDSDDEAVALVNGSDYGLAVAIHSASISRAQRMATHLNAGMVHINDQTVNNEFQVPFGGMGASGNGSRFGGPASFEEFSQTQWVSVMDQGIQYPF

SEQ ID NO: 138 - protein, 496 aa, Ideonella livida
MHTPATAGPLAADDTRRWSGRLYGAAGWQPAQGGTAAVTEKATGRALAEVALANAEDVDLAARSAAAAQTAWAATPFDQRAAVLRRAEALLAERAERFAHWNVREAGSIPPKAAWEWQATREQLSMAAALPMLPVGQVFPSAMLGRRNEWRRVPLGVVGVIAPWNFPLLLAMRSVAPALALGNAVILKPDLQTPVVGGQLIAELFEDAGLPAGVLQVLPGGPATGDALVRHPQVAMISFTGSTAVGRSIGATCGGLLKKCVLELGGNNALIVLDDADLDAAASSGAWGAFLHQGQICMQAGRHLVHRSVADAYAQRLAERAARLVVGDPAAGPVHLGPLVNERQAQKVAQIVDAAVAAGARVLAGGPREGLFFPATVLTGVTPDMAAFTEEIFGPVAPITVFDTEDELVALVHQSPYGLAAAIHTRHTPRGVALAQRLHTGMVHLNDQTVNNEFHVPFGGMGASGNGGRFGGPANVEEFTQTQWISVMEQGIQYPF

SEQ ID NO: 139 - protein, 487 aa, Burkholderia_sp._D7
MNDSKQARKWEGRIFSNGWVPAAGGTAPVIEPSTGDTLAAIGMGLPEDIDRAAHSASAAQPSWAAMPFDQRAAILREAARLLKEHASEINDWNVRECGSTRAKAEWELHATYEQLHMAAAMPMQPEGALFPSALPGRMNFCRQIPIGVVGVIAPWNFPLLLAMRSVAPALAVGNTVILKPDLQSAVAGGLLLAQVLEDAGLPAGVLHVVPGGPATGDALVRHPKVGMISFTGSTAVGRAIGQICGQMLKKVSLELGGNNAIVVLDDADVDAASSSGAWGAFLHQGQICMQTGRHLVHRSLAEQYASKLAERARKLAVGDPYKAQVHLGPLINQKQRDRIDDIVRKTLASGATLLTGGRFEKLFYQPTVLTGVTTDMPAFTEEIFGPVAPVTVFDDDDEAVALVNASDYGLAAALHTRSLSRGFALSSRIRAGMVHLNDQTVNNEFHVPFGGMGSSGNGGRFGGPANVHEFTQTQWISALDKPIAYPF

SEQ ID NO: 140 - DNA, 1458 bp, Hydrogenophaga aromaticivorans
  source 1..1458: mol_type = genomic DNA
aatactccggtgaaaacggagcgttggtctggcaaaatcttcaccggcagttgggtagccgcgagaggaggcgtggcccccgtactcgaagccgcaactggggcagccttaggggaagttggcgtggcaagtccggaagacgtggatgccgcagcacgcagtgcccaagctgcccagaaagcgtgggccgcaaccccgtttgatcaacgtgcggcgattgtgcgtgaagctgcgcgtctgctgaaagaacgcgcagcggagttcacccagtggaacgttcgcgaatgtggtagcattgtccccaaaggcgaatgggaagtggggatcacccacgaacagatgcagcaagctgcggcactggccggtcttccgaatggcatgatgttcccgtcgtcggtaccgggtcggactaacctctggcaacgggtaccgcttggcgttgtcggcgtcattgccccatggaactttccgctgtttctggccatgcgttcagttgctcccgcattggcgctgggcaatgcggtacttctgaaaccggatttgcagagcgcggttacgggtggggccctgattgctcgcttattcgaggatgtcggcttaccacccggtgtcctgcaggtgctgccaggcggcccagcgacaggtgatgctgtggtgaggcatccttgcgtcaacatggtcagcttcaccggatcaacagcggtgggacgtcagataggcgagttctgtgggcgtgcgttgaagaaggttgcactcgaactgggcggcaataacgccatgattgtgctggacgatgcggatttggacggtgcctcctcttgtgcagcgtggggcggttttctgcatcagggccagatctgcatggccgcgggtcgccatctcgttcaccgttctgtcgccgatgcgtatgccgcgaaattagtggaacgcgcgaaaaagctgtacgttggagatccgcatgcaggtcctgcgcatcttggccctctgatcaatgatcgccagacggaacgtgtgcatcgcattgtaaccgagtcgattgctgcaggcgcaaccctgctagctggcggtacccacgagggtcgcttctatcagccgacggttctgagcaatgtggcggttgacatgccagcgtttgctgaagagatctttgggccggtagctccgattaccgtgtttgacacggatgaagaagcggtcgcactggccaacagctccgaatacggtttagcggccgcgatccacagcaaatcgacagctcgagcgttgcgaatggcctcccaactgaaatcaggcatggtccacatcaacgaccagcctgtgaactgcgaacctcaagtgccgtttgggggtatgggagcgagcgggagtggtggtcgctttggaggtccggcttccattgacgagtttacgcaagcgcagtgggttagcgtttctgaaaaagcagcccagtatccgttc

SEQ ID NO: 141 - DNA, 1458 bp, Pseudomonas aeruginosa
  source 1..1458: mol_type = genomic DNA
cgcgaaacgaaagaacagcccatttggtacggcaaagtgttctccagcaattgggtggaagctcgtggcggcgtagccaatgttgtggatccgtcaaatggagacattctggggattacgggcgttgctaatggcgaagacgttgatgctgcggtgaatgcggcgaaacgcgcacagaaagaatgggcggcgattccgttttctgaacgcgctgcgatcgtgcggaaagcggcagaaaagctgaaggaacgggaacacgagtttgccgattggaatgtgcgagaatgtggtgcgatacgcccgaaaggtctgtgggaagctgggattgcctacgaacagatgcaccaagcggccggactggcgtatctgtcgaacgggaccttgtttcctagtgcggtgcctggcaggatgaacctgtgccaacgtgtcccagtgggtgttgttggggtcatagcgccttggaacttcccgttgtttctggcgatgcgttcagtagcaccagcgctcgccttgggcaatgccgtgatcctgaagccggatctgcagacagccgttactggtggcgcactgattgccgagatcttttccgatgccggtatgccagatggcgtgctccatgtgttaccagggggtgcagatgttggtgagagcatggttgccaactctggcatcaacatgattagcttcaccggctctacgcaggtgggccgtctgattggcgagaaatgcggtcgtatgcttaagaaggtggcgttggaactgggtgggaacaatgtccacatcgtgttacctgatgcggaccttgatggcgcagtttcgtgtgcagcatggggcacctttctgcatcagggtcaggtttgcatggcagcgggccgccatctagtccatcgtgatgtggctcagcagtatgctgagaaacttgctttacgtgcaaaaaacctcgtcgtcggtgacccgaacagtgatcgcgttcatctgggtccgttgattaacgacaaacaggtagtacgtgtccacgcactcgtggagagcgctcaatcagcaggcgcaaaagtactggccggagggacctatcaggatcgctattaccaagctaccgtcattatggatgtcaaaccggaaatggaggtcttcaaatccgaaatcttcggtccggtagcgcccatcacagtgttcgacagcattgaagaggccattgaactggccaattgcagcgaatatggccttgccgcgtctatccatactagagcgttagcgacgggcttagatatcgcgaaacgcctgaacaccggaatggtgcacattaacgaccaacccatcaactgtgaaccgcatgtaccgtttggagggatgggctcatccggctcgggtggtcgctttggtggtctggccagcattgacgaattcacccaaagccagtggatcagtatggttgagaaatcggccagttacccgttt

SEQ ID NO: 142 - DNA, 1458 bp, Pseudomonas sp. MAP12
  source 1..1458: mol_type = genomic DNA
catgaaaccaaagaacagccaatatggggaggcaagatcttctcgagcacctgggtagaagcgcgtggtggtgtagctaacgtggtggatccctctaatggagacatcctgggcattactggcgttgcaaaccgcgaagatgtggatgtggctgtttccgcggccaaaattgcccaaaaagaatgggcagcgatgccgttttccgaacgcgcagcaattgtgcgtaaagctgccgacaaactgaaagagcgggaacacgagtttgccgattggaatgtccgcgaatgtggggcgattcgtcccaaaggcttatgggaagcgggtattacgtacgaacagatgcaccaagccgttggccttgcctcactgccgaatggtgccctgttccctagtgccgttagtggccgcatgaatctctgccagagagtcccgattggggttgtcggtgtgatagccccgtggaattttcccctgtttctggccatgcgaagcgtagcaccagcgttggttctgggcaatgcggtggtgctgaaagcggacttgcagacagccgtgattggaggtgccctaatcgctgagatcttttcagatgcgggtattccagaaggagttctgcatgtacttcctggcggtgcagacgttggcgaatcaatggtcgagaatcctggcatcaacatgatctcgttcacggggtctactcaggtcggtcgctccattggcgaaaagtgtgggcgcatgttaaagaaggtgagtctcgagttaggcggtaacaacgtcaacattgtcctcccggatgcggatcttgatggcgcagtgggttgtgcggcgtggggtaccttcttccatcagggtcaggtgtgcatggcagcgggtcgccatctggtccatcgtgatattgcgcaggaatatgcagccaaactggcgaaacgggcgcagtcactggttgtaggggatccgaacaccgaccaagtgcatctgggccctttgatcaacgacaaacaagttgatcgtgttcacgctctggtggaatctgccgaacgtgcaggtgctaaagtcctggcaggtggcgcgtatgaaggtcgctactatcaagccaccgtagtgatggatgtcaaaccggacatggagattttccagagcgagatctttggcccggttgccccaatcacgattttcgacagcattgatgaagctatcgaattggcgaattcgtccgaatatggcttagcggctagcatccacacgaaatcgctcaccaccgggatgaagatcgcgaatcgtctgaaaacgggtatggtgcacattaacgatcaaccgatcaactgcgaaccgcatgtaccgtttggcggcatgggggcatctggcagtggaggacgttttgggggcactgctagcatcgaggagtttacccagagccagtggattagcgtggtggacaaaacagcggtttacccgttt

SEQ ID NO: 143 - DNA, 1464 bp, Alteromonas
  source 1..1464: mol_type = genomic DNA
caacaggaacgtaagaaggaagtgccgatttggtcggggaaagtcttctcctcagggtgggtggaagcgcgtggtggcgcgtctgatgtgaccgatccgagcaacggtgatctcctgggcgtggtgggcattgcgaatggcgaagacgttgccgcggccgcacagagtgctcgcagagcgcagaaagaatgggctgcgattccgtttagcgaacgcgccgaaattgtcaggaaagcggccgaaaaactgaaagaacgcgaaaatgagttcgcggattggaacgttcgggaatgtggtgcgatccgccagaaaggcctgtgggaagctggtatcacctatcagcagatgcaccaagcggcaagtctcgcttttctcccagatgggacgagtttaccctccactgtggctggtcgcctgaacttgtgccatcgtgtgccggttggggtagtaggcgtcattgcgccgtggaattttccgctgttccttgcgatgcgatccgtagctccagcactagtactgggcaatgcggtcattctgaaaccggatcctcagactgccgttacgggtggtgcattgattgcggagatcttctctgaagccggcattcctgatggtgtgatccatgtgctaccaggaggagcggaagctggcgaatcgatggtaaccaatccggggattgacatgatctcgttcacagggagcacagaagtcggacgcttaatcggggagaagtgtggacgtatgctgaagaaagtggcactggagttaggcggcaataacgtccacatcatcctgccggatgcagacctggatggcgcagcgtcttgtgcagcctggggtacctttctccatcaaggccaggtttgcatggcagcgggtcgtcacttagtccaccgtgacatagcccaggaatatgcggagaaactggcactgcgtgcccgtaacctggttgtcggtgatcccaaaacggaccaggttcatcttggcccgttagttaacgacaaacaggtggcgcatgtgcatgctctggtggagagcgcccaaaaagccggcgcaaaaattctggctggtggaacttaccaagatcgctattaccaagcgaccgttcttatggatgtcacccctaagatggacatcttcgagttggaaacgtttggtccagttgccccgattaccatcgttgactctgtggaagaggccattggcctggccaattcgagcgaatacggtttggcagcaagcatccacacgaaagatcttgctgcgggtttggagatagcccgcaacctgaaaacaggcatggtgcacattaacgatcagccgattaactgcgaaccacatgtaccctttggtggcatgggtgcctcagggtcatccggccggtttggaggcctggcgagtatcgacgcgtttacccaaagccagtggattagcatggtgggcaaacctgccacctatccgttt

SEQ ID NO: 144 - DNA, 1458 bp, Tepidiphilus succinatimandens
  source 1..1458: mol_type = genomic DNA
aactggaatggcaaattgccgatatggcatggcaaagtgttctccaatgggtgggtcgttcctagaggtggagttgcggacgtagtggatcccagtagtggcgatgtactgggtgttaccggcatagcgaacagcgaagatatcgctaccgccgcatctgcggcgaaagaagcccagaaaaagtgggcggccatgccgttcaatgatcgagcggccattttgcggaaagccgccgaaaaactgcgtgaacgcgaagcggaattcgcagattggaatgttcgcgagtgcggtgctgtacgcatgaaaggcgtgtgggaagcggggattacctacgaacagatgcaccaagctgcgtcgctagcctttctccctaatggaacgttgtttccatcacaggtgccaggccgtatgaactttgtgcatcgcgttccggtgggtgttgtgggcgtgattgccccgtggaattttcccctgttcctggcgatgcgcagcgttgcaccagcattggttcttggaaatgcggtcattctgaagcctgacgtccagacagctgtgaccggtggtgcgctgatcgcagagatctttgcagaagcaggcattccggaaggtgtcttacatgttctcccgggtggtgccgatgcgggcgacgcgatggtcaccaatccggagattgacatgatttccttcactggcagcactgctgtgggtcgtcagattggcgagaaatgcggccgtatgctgaagaaggtgacgctggaactgggtgggaacaacgtgcacattgtcctgccggacgccgatctgaccggtgcagcttcgtgtgcagcatgggggacgtttctgcaccaagggcaggtttgtatggctgctggccgtcatctggtgcaccgcgatgttgcccagcaatatgcgcaggagttagccgcacgtgccaaaaacctcgtagttggcgatcccaaaaccgatcaggtccatcttggcccgctgatcaacgacaaacaagtcgctcgcgtgcatgcgcttgtcgaaagtgcgcagaaacaaggtgcgaaagtgctcgtaggagggacgcatcaaggccgcttttaccagccaacagttctgatggatgtacgtccggacatggacgtcttcaagtctgagatcttcggtcctgtggcaccgatcaccgtgtttgatacgattgatgaggcgatcgaactggccaatagcagcgaatatggcttagcggctagcatccatacctccgcaattgccactgcgcttcaaattgccaaacggctgaaaacaggcatggtgcacatcaacgatcagccgattaactgcgaaccacacgtaccgtttggcgggatgggtgcgtcaggtacttcgggtcgttttggcggattatcgtcaatcgacgaattcacgcagagtcagtggatctctatggtcgaaaaacccaccaactatccgttt

SEQ ID NO: 145 - DNA, 1458 bp, Halomonas cupida
  source 1..1458: mol_type = genomic DNA
tcgacctttttcaacgcggaaacgtacagcaatcgcatctacctgaatgattggcgggaaagtcgcggtggtacaagcgatgtggtggaaccggcgacaggcaaagtcctggcgagaaccgctattgggaactccgaggatatccgggaagcgattgtggaagccaaagctcagcaaccggcatgggcgaggttacccttcgaccaacgagcccgcattctgcgccgtgccgctgaattgttgctggaacaccgtgacacctttatcgaatggaacatccgcgaatgcggctctatagtcccgaaagcggaagccgaacttcactcgacgcacgaacagctgaacatggcggcggctatgactatgcagccagatggcattaccctgccgtcaagcatgcctggtcgccgtaatacctgtcgtcgagtgccgttaggcgtagtcggagtcatcacaccgtggaactttccgttgctgctggccatgcggtccgttgcgccagcaattgccgttggcaatagcgtggttctgaaaccggatcatcagagcgcagtgaccggtggtttgctgattgcccgcttattcgaggaagcgggcttaccggccggggtactgcaagtcattcccggaggcgcggaagcaggtgaagcccttgtgacgcatccactcaccgccatgatctcctttactgggagtactgcggtaggtcgcaaaatcgggcgtacatgtggggagctgctgaagaaaagtgcccttgaactgggtggcaataacgcgttcattgtgctggatgatgccgacattgatgcggcagcatcccatggtgcttggggagcctatctgcatcaaggccagatatgcatgcaatcaggccgtcactttgtccaccattctgtcgctgaggcgtatatcagcaagttagctgaacgcgcagaacgccttaccgtggcggatcccttcttaggcactgcagacatcggcccgctgattaacgcgcaacagctcgagaaactggatatggccgttacggcgtcaattaacgacggagcccgtctagttacgggtggtcattcccatggacagttctatcgtccgacggtgctgagcaatgtgtcgattgatatgccagcgtttcagcaggagctctttggcccagtagcaccggttaccacctttcatgacgaagaagagctgatcgagaaagtgtctgcttcatcgtatggcctagcagcggcaatccattcgagctctattggtcgtgcgttggatctcgccgagcgtattccggctggcatgattcacatcaacgaccagaccgtaaataacgagttccaggttccttttgggggttttggtgatagtggcaatagtggccgctttggtggccctgcaaatctggaagaattcacgcaaagccagtgggtttctttgatgaacactccgcgtacctaccctttc

SEQ ID NO: 146 - DNA, 1491 bp, Pseudomonas fluorescens
  source 1..1491: mol_type = genomic DNA
accaccgctaacctgcacaaccagtacccgtcgattgccgagttcatcgcggaacaccgttggaaagcgtgcttttatccgggtgcctgggaaagtgccgaacgtgagatccccgtttttgagccagcaacgggtgagcgtctagcgagcgtcggaattgctagtgcagccgaagtagctagggcgggattgcgcgcacgccaagcgcaaccagcatgggcagccaccccatttgaccagcgtgcggcgatcttacgcgaagcagcgcgtcttctgcaacaggaagccgaaagcttcatcgagtggaatatccgggaatgcgggggtgcccgtttcaaagccgaatgggaactcaacatatgcgtagagcagctgcagatggctgctgcaatgcccatgcaagccaatggggaacttttcccgtccagcatgccaggacgcaccaacatttggcgaagagtgccgatgggagtagtggcggtgattagtccgtggaactttccgctcctgttgtcgttgcgctccattgcccctgctctcgcacttggcaatgccgtcttgctgaaaccgtcagagttcagctctgtgactggcggtctgctgttagcgcgtctgtttgagctggctggcgttccgcaaggtgtctttcaggtcttacctggtttagccgaaacgggttctgccctggtatcggatccctgcgtcaaaatggtggcatttacgggctcaacagcggttgggcgccgcattgcagaaacttgtggcggcttactgaaacgctgttccctggaactgggtggtaacaacgcgctgattgtgtgtcccgatgcggaccttgatgctgcctccagttctggcgcatggggcagcttcctgcatcagggccagatttgcatgcaggcgggccgccacattgtgcatcgaagcgttgttgctgcctacacggaaaagctgaaagatcgcgcggaacgtctggcgtgtgggaatccttttaccgaagcggtacaactgggtccgctgattaatgcacagcaacgcgatcgggtccatggtttggtccaggatgcggtgcatcaaggcgcgacgttggtgacagggggtgagtacaaagaactctgctatcgccctaccgtactgataggcgtgactccggatatgccggtcttcaaggacgaaatctttggcccagtggcgcctatcgttgtgtatgatgacatcgaagaagctctggcgctagtgaatgcgagcccgtatggcttagcagtggccattcacaccggcaatgccacacgtggttacgaatgggcaggccgtatccattcgggcatggttcatgtgaacgaccagacggttaacaacgagttccaggttccgttcgggggtatgggcgcctcaggttacggaggccggtatgggggtccggcgaattttgacgagtttaccgaacgtcagtgggtttctctgaccagcgatccgattcagtatccgttt

SEQ ID NO: 147 - DNA, 1458 bp, Glaciimonas immobilis
  source 1..1458: mol_type = genomic DNA
aacaccagtaccgtaacgaacatttgggacagcaagatctactcaggcggttggattgccgccgaaggcggaactgccgccatcattgaaccggcaacagaacaggtgctgggacacattggcatcggcgcaactcaggacgttgatcgcgcggtgcagattgccagtcatgcccagaggtcttgggcgcgtatgccgtttgaccaacgcgcgaacattatgcgggaagctgcgcgtttagtgctggagagagctgcggagttcaatgtgtggaacattcggcaatgcggatctatccccgctaaagcggagtgggaactgcatgctacctgtgagcagattctcatggcagctgcgttaccgatgcaaccggaaggcttgctgtttccgagcagcatgccagggcgcacgaacctgtcgcgtcaactgccgattggcgtgataggcgtgatcaccccttggaactttccgctgctgctggccatgcgctcggtagctcctgccttagcactgggtaatgcggtgatccttaaaccggatcaacagagtgccatttgtggtggtgcactcattgctcaagctttcgaagatgcaggccttcctgtgggcgttctgcatgtgattccaggcgggccggccactggcgatgctctagtgaaacatccggaagtcggcatgatttcgtttaccggttcaaccgcggtcggtcgagcgattgggcaaacgtgtgggtacctcttgaagaaagtggccttagaactggggggtaataacgcgatcatcgtcttggatgatgcggatatggatgccgcgtcttccaatggggcgtggggtgcattcctgcaccagggccagatttgcatgcagacaggtcgtcatctagtccatcactccgttgccgaccagtatgcagagaaattggcggctcgtgcggaaaaactgcacgtaggcaatccccataccgatcaagtgcatctgggtccgctgattaaccgcaaacagtgcgaccgcatccacggtatcgtccaggaaacccttcgtgcgggcgcacatgcactgaccggtgccacccatgaacgcctgttctatcgtccaacggttttaacgggcgtaacaccggatatggcagcgtttcaggaggaactgtttggcccagttgcgccagttacggtattccacgatgatgacgaagccgttgaactggttaatcgtagtgcctatggcctttgcgcagcaatccattcgcgcaacataccccgtgcggtggcgttgtcccagcgcctcaatacgggtatgatccacattaatgaccagaccgtcaacaacgagttccacgttccctttggaggcatggggagctcaggcaacggtggacgctttggtggtccggcgaatgtccacgaattcactcagagccaatggctgagcatcatggaaaaaccggtcatctaccctttt

SEQ ID NO: 148 - DNA, 1458 bp, Paraburkholderia unamae
  source 1..1458: mol_type = genomic DNA
acggggactggcagcgaaggccaatggaccggcaagatcttcctgggcgaatgggtcaaaggaacgggtgcaacagccccggtgatggagcctgctacagacaatcagattggtaccattgccctggccagtcgagaagacgtggacacagccatagagcgcgcagtggttgcgcagcgtgcctgggctgagacgacgtttgacaaacgagcggcagtgttgcacgaagcggcacgcctgattaaggcccgtgcagaacgcttcaactactggaacgtgcgcgaatgcggcagcatcgtgccgaaagcgcagtgggaactggatgccagctatgaacagctactgatggctgctgcgttaccgatgcacccgactgggacgttattcccctcaagcatgccaggtcgcaccaatacctggcgccgcttaccgattggtgtcgtgggcgtaattgcgccgtggaactttccgctgctcttggcactgcggtcagttgcaccggccattgcactgggcaatgccgtcgtcctgaaacccgatcagcagagtgcggtgactggtggcgcactgatcgcggaactgttcgaagatgccggtcttcctcgtggcgtgctgcaggtgttacccggtggggcccagaccggtgatgcggtagtccgtcatccggcagttgggatgatcagcttcactggatctaccgccgttggtcgccaaatcggcgaaacctgtgggcgcatgctgaagaaaaccagtttggaactgggtggcaataacccgattatcgtgcttcctgatgctgatctcgataaagcggcatcatgtgccgcatggggcgcgtttttgcaccaagggcaaatctgcatgcaagccggcaggcatctggtgcatcgctctgttgcggaaagctacgtggctaaacttgcggctcgtgcccggaaactcgcggttggaaacccagcgaccgaacccgttcacattggtcctctcattaatgcgagacaggcagaacgcgtcgaacggatagttcgtgattccgtcgaaatgggcgctgtaattgccgcggggggacaacgtcgtggtcgctttttcgaaccgacagttctggcggatgtcaccccgcatatgccagcgtttaaagacgagatttttggaccagtagctccggtgacgctgttcgattccgtagacgaagccatcgagttagtgcatgcctcggaatatggccttgcagcggcggtgcattcgggctctatgagtgcggcgatgtcggttgcacgtcgtctgaaatccggtatgatccacattaacgaccaaacggttaacaacgagttccaggtaccgtttggcggcatgggtgcttcgggtaatggcggccgttttggtggtccagcgaatgtcgaggagtttacccagacccagtggatcagcgctatggatgcccctattgagtatccgttt

SEQ ID NO: 149 - DNA, 1455 bp, Marinobacter salsuginis
  source 1..1455: mol_type = genomic DNA
gatatgccagctagcccagtatggcaagagcagctctttttaggctcctggaaaagtggggatggtgatcagatcaacgtagtggaacctgcaacaggtgcggtcatctcgaagctgaagatagcgaccgcaggggatgtggaacgcgcagcaacgattgcacgcgacacccagactgcgtgggctatggtgccgttcgatcagaaagcggaaatcctccgcaaagcggcggcgctgctgaaagagagagccaacgagatcaatgactggaatacgcgggaatgcggttcggtaggaccgaaagcggactgggaactgcaagcgacctatgaacaggcccagatggctgcagcattgccgatgcagccgaatggcgaaatcttcccatcaaacatgcccggcaaacgcaactattggaaacgtgtccccattggtaccgtgggtgttattgcgccatggaatttcccgattctgctcgcgatgcgtagcgtgttcccagctttggccatgggaaatgccgtgattctgaaaccggatcccaagagctccatttgtggcggtgctcttatggcccagattctgagcgatgcaggcttaccggaaggcgtgttccacgttctgcctggtggcccggaagttggccaagcgttagtggaacatccgctggtgaaaatgatttcctttacgggctctactgcggtcggacgcaagatcggcgaaacatgcggtcgaaccctgaaaaaagcggctctggaattgggtgggaacaatgcccaagtcgttctggaagatgccgaccttgacatcgctagtagctgtggtgcctggggcgcctttctgcatcaagggcagatttgcatgcagactggtcgtcacctagtgcatacgtcggttgccgaggaatacttgagccgtcttgccagtcgcgcagaaaacctggcctgtggtaatcctgcacaggaacaagtgcatcaggggccgctgattaatggcgttcaggccaaacgggtagaggatattgtcaatcgctcagtagagatgggagcacgcatagtcactggtggcaaacgtcatggcaactactacgaaccgaccgttatcaccgatgtgacctccaacatgccggtttttagcgaggaagtgtttggcccggttgccccggtgatgaccttcgacagtgattcggaggcttgcgaactggtgaacgaatctccctatggcttagctgcggcgattcacagtggttctacggagcgtgcgctcaaaatcgcgaaccgtatccaagtcggcatgattcacattaacgaccagacggtaaacaacgagtttcaggttcctttcggaggtatggggtcgtcagggaattctggccgttttggtggccctgcgaatatcgaagagtttaccacatcacaatggatcagcgtcatggaagaaggcattcagtatccgttt

SEQ ID NO: 150 - DNA, 1455 bp, Aromatoleum toluclasticum
  source 1..1455: mol_type = genomic DNA
aacgatcgcaatactacgcgctggcatcaacgcatctttgtaggcgaatggacaccgggtcgtggtgacacggttccggtgattgagccagctacgggcgatcaactggcgctgctcagtaccgcgtcgattgaggatgttgatgcagcagcgcgtctagctgccgaagcacagccagcttgggcggcactgccctttgatcgtcgcgcagcagtcctgcgcaaagttgcccaactgctgcaagaacgcgcagcggaaatcaaccactggaacatccgtgaatgcggcagtattccgccgaaagcggaatgggagctgaatgcaaccatcgaacaggcccatatggccgcagccatgcctatgcagccgattggtgagatctttccctcgagcatgcctggtaggcgcaactactggcagcgtctgcctattggtgtggttggcgtcattgccccctggaactttccgatcttgctgggccttcgcagcgtattgccggcgttagctatggggaatgcagtcattctcaaaccggacttacagagcgcgatttgcggaggcctgttgctggccgaagtgttcgaagatgctggcctgcctaaaggggtcttccacgtactgccgggtggcccagttacgggtgatgccctggtgcgtcatccccgtgtcaagatgatcagctttaccggtagtaccgcggtcggccgcttgattggcgaaacctgtggtcgtatgctgaagaaggtagcgctcgaactgggcgggaacaatgccatggtcatacttgacgatgctgatcttgaaagcgcctcttcctgtgctgcatggggcgcgtttctgcatcaagggcagatttgcatgcaggctggtcgtcatttagtgcatcgcaaagtagccgaccgctatgccgagttgctggcagtgcgtgcggctaaactggtggttggtaatccggcgacaggtccggtgcacttagggccgttaatcaacgatcggcaagccgcgaaagttgcagaagtcgtagaacggtcagcggcgttaggtgcgcgagtgctagcgggtggaaaacgtgatggccggttctttccggccactgtgcttgcaggagttaccccagatatgccggcttatacggaagaaatcttcggcccagtggcgccgattaccgtgttcgactctgacgacgaagcggttgcgctggtcaatggatccgattatggcctggctgttgccatccattccgccagtatatctcgagcgcagagaatggcgacacacctcaacgccggaatggtgcacattaacgaccaaaccgtgaataacgagtttcaggtgccgtttgggggcatgggtgcgtcaggcaatggctcacgctttggcggtcctgcctcgttcgaggagttctcgcagactcagtgggttagcgtgatggatcaggggattcagtacccattc

SEQ ID NO: 151 - DNA, 1485 bp, Ideonella livida
  source 1..1485: mol_type = genomic DNA
catactccagccactgcgggcccactggctgcggacgatacgaggcgctggagtggtcgcttgtacggtgcagcagggtggcagccggcgcaaggtggtacggctgctgtgaccgagaaagccacaggccgagccttggcggaagtagctctggctaatgcggaagacgtcgatttagcagcacgtagtgctgcagctgcccagacggcatgggcagcgactccgtttgatcagcgtgcagcggtccttcgccgtgcggaagccctgttagccgaacgcgcggaacgtttcgctcactggaatgtgcgtgaagccggctcgattccccctaaagcggcttgggaatggcaagcgacacgggagcaactcagcatggcggctgcactaccgatgctgcctgtaggccaggtttttccgtccgcgatgctggggcgccggaacgagtggcgtcgcgttccattgggcgttgtcggggtcatcgcaccctggaactttccgctgctgctcgccatgcgttcggtggcaccggcccttgcgctgggaaatgccgttatcctaaaaccggatcttcaaaccccagtggttggcggtcagctgattgccgagctgttcgaagatgccggtctgccggctggtgtgctgcaggtattgccggggggcccagcgaccggtgatgccctcgtccgtcatccccaggttgcgatgattagcttcaccggctctaccgccgtcggtagatcaattggggctacctgtggcggcctgctgaagaaatgcgtgcttgaactgggcggcaacaatgcgctgattgtcctcgatgatgccgacctggatgcagcggcctctagcggagcgtggggtgcgtttctgcaccagggccagatctgcatgcaagcaggtcgccatctggtccatcgatcggtagccgacgcgtatgcgcaacgtcttgcggaacgcgcagcacgtctggtagttggcgatcctgccgccggtccggtgcatctcggaccgttagtcaacgaacgtcaggcgcagaaagttgcgcagatagtggatgccgcggtagctgcgggtgcacgtgtgttagcgggaggtccacgcgaaggcctgttcttcccggccacagtgttaaccggagttaccccggacatggcggcgtttaccgaggagatctttggaccggttgctcccatcaccgtgtttgatacggaagacgaattggtggccttagtgcatcagtccccgtatggtctggcggcagcaattcacacgcggcacacacctcgcggtgtggcattggcgcaacgcctgcatacgggcatggttcacctgaacgaccaaactgtgaacaacgaattccacgtaccgtttgggggcatgggcgcctcagggaatggcggtcgctttggcggccctgccaatgtggaggaattcacccagacgcagtggatcagcgtcatggaacaagggattcagtacccgttt

SEQ ID NO: 152 - DNA, 1458 bp, Burkholderia_sp._D7
  source 1..1458: mol_type = genomic DNA
aacgacagcaaacaggcacgtaagtgggaaggccgcattttcagcaacggttgggtgccagcagcaggtggcactgcccctgtgatcgaaccttcgaccggtgatacgttagcggcgatcggcatgggcttaccggaggatattgatcgtgcagcccattcggctagcgccgcccaaccgagttgggctgcgatgccgtttgaccagcgtgccgccattctgcgtgaagccgcgcgcttactgaaagaacatgcgtccgaaatcaacgattggaatgtccgcgaatgtgggtctacgcgcgctaaagcggaatgggaacttcacgcaacgtatgagcagctccacatggcggccgcaatgcccatgcaacccgaaggcgctctttttccttcggcactgccaggacgcatgaacttttgccgccaaattccgattggcgttgttggcgtcattgccccgtggaacttcccgctcctgttggccatgcgctcggttgcgcctgccctggcggtgggtaacaccgtcatcctgaaaccggatctccagtctgcggtggcgggaggcctactgcttgctcaggttctggaagatgccggtcttccagcaggtgttctccatgtggttcccgggggaccagctacaggggatgcgctagtcagacatccgaaagtgggcatgatcagctttacgggcagcactgcggtaggccgggcaattgggcagatatgtgggcagatgctgaagaaggtaagcctggaactgggtggcaacaatgcgattgtcgtgctggatgacgcggatgttgatgccgcgagtagttcaggcgcttggggagcgttcctccaccagggtcagatctgcatgcaaaccgggcgacatctggtgcatcgtagcttggcagaacagtacgcttcaaaactggccgaacgtgcgcgcaaattggcagttggcgatccgtacaaagcccaagtccacttaggtccgctgatcaaccagaaacaacgcgacaggatcgatgacatagtacgcaaaactctggcatcaggtgcgactctgctgacaggtggtcgtttcgagaagttgttctaccagcctaccgtattaacgggggtaaccacagacatgccggcgtttaccgaggagattttcggtccggttgctccggtaaccgtgtttgacgatgacgatgaagcagtggcgttagtcaatgcctccgattatggtctggcagctgcgttgcatacccggtcactgagtcgaggctttgcgctgtcctcccgtattcgtgctggcatggtgcacctgaatgatcaaaccgtgaacaatgagttccacgtgccctttggaggtatgggctctagcggcaatggcggtcgttttggtggcccagcgaatgtccatgagttcacccagacgcagtggatttctgccttggacaaaccgatcgcctatccgttt

SEQ ID NO: 153 - DNA, 30 bp, synthetic construct
  source 1..30: mol_type = other DNA
caccatcacggatccaatactccggtgaaa

SEQ ID NO: 154 - DNA, 38 bp, synthetic construct
  source 1..38: mol_type = other DNA
cagctaattaagcttttagaacggatactgggctgctt

SEQ ID NO: 155 - DNA, 30 bp, synthetic construct
  source 1..30: mol_type = other DNA
caccatcacggatcccgcgaaacgaaagaa

SEQ ID NO: 156 - DNA, 39 bp, synthetic construct
  source 1..39: mol_type = other DNA
cagctaattaagcttttaaaacgggtaactggccgattt

SEQ ID NO: 157 - DNA, 30 bp, synthetic construct
  source 1..30: mol_type = other DNA
caccatcacggatcccatgaaaccaaagaa

SEQ ID NO: 158 - DNA, 40 bp, synthetic construct
  source 1..40: mol_type = other DNA
cagctaattaagcttttaaaacgggtaaaccgctgttttg

SEQ ID NO: 159 - DNA, 30 bp, synthetic construct
  source 1..30: mol_type = other DNA
caccatcacggatcccaacaggaacgtaag

SEQ ID NO: 160 - DNA, 39 bp, synthetic construct
  source 1..39: mol_type = other DNA
cagctaattaagcttttaaaacggataggtggcaggttt

SEQ ID NO: 161 - DNA, 30 bp, synthetic construct
  source 1..30: mol_type = other DNA
caccatcacggatccaactggaatggcaaa

SEQ ID NO: 162 - DNA, 40 bp, synthetic construct
  source 1..40: mol_type = other DNA
cagctaattaagcttttaaaacggatagttggtgggtttt

SEQ ID NO: 163 - DNA, 30 bp, synthetic construct
  source 1..30: mol_type = other DNA
caccatcacggatcctcgacctttttcaac

SEQ ID NO: 164 - DNA, 38 bp, synthetic construct
  source 1..38: mol_type = other DNA
cagctaattaagcttttagaaagggtaggtacgcggag

SEQ ID NO: 165 - DNA, 30 bp, synthetic construct
  source 1..30: mol_type = other DNA
caccatcacggatccaccaccgctaacctg

SEQ ID NO: 166 - DNA, 39 bp, synthetic construct
  source 1..39: mol_type = other DNA
cagctaattaagcttttaaaacggatactgaatcggatc

SEQ ID NO: 167 - DNA, 30 bp, synthetic construct
  source 1..30: mol_type = other DNA
caccatcacggatccaacaccagtaccgta

SEQ ID NO: 168 - DNA, 40 bp, synthetic construct
  source 1..40: mol_type = other DNA
cagctaattaagcttttaaaaagggtagatgaccggtttt

SEQ ID NO: 169 - DNA, 30 bp, synthetic construct
  source 1..30: mol_type = other DNA
caccatcacggatccacggggactggcagc

SEQ ID NO: 170 - DNA, 39 bp, synthetic construct
  source 1..39: mol_type = other DNA
cagctaattaagcttttaaaacggatactcaataggggc

SEQ ID NO: 171 - DNA, 30 bp, synthetic construct
  source 1..30: mol_type = other DNA
caccatcacggatccgatatgccagctagc

SEQ ID NO: 172 - DNA, 39 bp, synthetic construct
  source 1..39: mol_type = other DNA
cagctaattaagcttttaaaacggatactgaatgccttc

SEQ ID NO: 173 - DNA, 30 bp, synthetic construct
  source 1..30: mol_type = other DNA
caccatcacggatccaacgatcgcaatact

SEQ ID NO: 174 - DNA, 39 bp, synthetic construct
  source 1..39: mol_type = other DNA
cagctaattaagcttttagaatgggtactgaatcccctg

SEQ ID NO: 175 - DNA, 30 bp, synthetic construct
  source 1..30: mol_type = other DNA
caccatcacggatcccatactccagccact

SEQ ID NO: 176 - DNA, 39 bp, synthetic construct
  source 1..39: mol_type = other DNA
cagctaattaagcttttaaaacgggtactgaatcccttg

SEQ ID NO: 177 - DNA, 30 bp, synthetic construct
  source 1..30: mol_type = other DNA
caccatcacggatccaacgacagcaaacag

SEQ ID NO: 178 - DNA, 39 bp, synthetic construct
  source 1..39: mol_type = other DNA
cagctaattaagcttttaaaacggataggcgatcggttt

SEQ ID NO: 179 - DNA, 39 bp, synthetic construct
  source 1..39: mol_type = other DNA
aagaggagaaattaactatgcgtgagaccaaggagcaac

SEQ ID NO: 180 - DNA, 41 bp, synthetic construct
  source 1..41: mol_type = other DNA
aagctcagctaattaagcttttacgcttcttcgacacttac

SEQ ID NO: 181 - DNA, 25 bp, synthetic construct
  source 1..25: mol_type = other DNA
catagttaatttctcctctttaatg

SEQ ID NO: 182 - DNA, 22 bp, synthetic construct
  source 1..22: mol_type = other DNA
aagcttaattagctgagcttgg

SEQ ID NO: 183 - DNA, 40 bp, synthetic construct
  source 1..40: mol_type = other DNA
aagaggagaaattaactatgaacaggttaccttcgagcgc

SEQ ID NO: 184 - DNA, 22 bp, synthetic construct
  source 1..22: mol_type = other DNA
ggtatatctccttcttattacg

SEQ ID NO: 185 - DNA, 41 bp, synthetic construct
  source 1..41: mol_type = other DNA
taagaaggagatataccatgatcataggggttcctaaagag

SEQ ID NO: 186 - DNA, 40 bp, synthetic construct
  source 1..40: mol_type = other DNA
catggtatatctccttcttattaagcacccgccacagatg

SEQ ID NO: 187 - DNA, 44 bp, synthetic construct
  source 1..44: mol_type = other DNA
taagaaggagatataccatgacgaatactctggatgttttaaaa

SEQ ID NO: 188 - DNA, 20 bp, synthetic construct
  source 1..20: mol_type = other DNA
ttaagcacccgccacagatg

SEQ ID NO: 189 - DNA, 22 bp, synthetic construct
  source 1..22: mol_type = other DNA
taagaaggagatataccatgac

SEQ ID NO: 190 - DNA, 36 bp, synthetic construct
  source 1..36: mol_type = other DNA
gtggcgggtgcttaataagaaggagatataccatgc

SEQ ID NO: 191 - DNA, 20 bp, synthetic construct
  source 1..20: mol_type = other DNA
cacttattcaggcgtagcac

SEQ ID NO: 192 - DNA, 22 bp, synthetic construct
  source 1..22: mol_type = other DNA
atcggcattttcttttgcgttt

SEQ ID NO: 193 - DNA, 20 bp, synthetic construct
  source 1..20: mol_type = other DNA
ccaattgacttcggcaagtg

SEQ ID NO: 194 - DNA, 43 bp, synthetic construct
  source 1..43: mol_type = other DNA
gtgctacgcctgaataagtggggttattccttatctatctaat

SEQ ID NO: 195 - DNA, 43 bp, synthetic construct
  source 1..43: mol_type = other DNA
acgcaaaagaaaatgccgatgaggtaaaagaataatggctatc

SEQ ID NO: 196 - DNA, 20 bp, synthetic construct
  source 1..20: mol_type = other DNA
gtcgcgtgaacataagcgtc

SEQ ID NO: 197 - DNA, 46 bp, synthetic construct
  source 1..46: mol_type = other DNA
gatagccattattcttttacctcgggttattccttatctatctaat

SEQ ID NO: 198 - DNA, 46 bp, synthetic construct
  source 1..46: mol_type = other DNA
attagatagataaggaataacccgaggtaaaagaataatggctatc

SEQ ID NO: 199 - DNA, 20 bp, synthetic construct
  source 1..20: mol_type = other DNA
ttaaaacgggtagttcgccg

SEQ ID NO: 200 - DNA, 38 bp, synthetic construct
  source 1..38: mol_type = other DNA
aactacccgttttaataagaaggagatataccatgatc